European Patent Specification EP 3 710 568 B1, published July 17, 2024. Title: METHOD OF CLEANING A SURFACE HAVING SOIL COMPRISING FATTY ACID AND CONSUMER PRODUCT COMPOSITION THEREFOR. Applicant: The Procter & Gamble Company Velasquez, Juan E. Gonzales, Denis A. Bettiol, Jean-Luc P. Geary, Nicholas W. The sequence listing filed with the application follows.

SEQUENCE LISTING (80 sequences)

SEQ ID NO: 1 - protein, 1165 aa, Gaeumannomyces graminis
MTVSTHHDDSPGLSGRLRDLLHHVFGNQKSPTVYPNAPGNSAKPVPTGLADDIDKLGFKDIDTLLIFLNSAVKGVNDDQQFLLEKMIQLLAKLPPASREGKKLTDGLINDLWDSLDHPPVASLGKGFSFREPDGSNNNIHLPSLGAANTPYARSTKPLVFQNPNPPDPATIFDTLMVRDPAKFRPHPNKISSMLFYLATIITHDIFQTSPRDFNINLTSSYLDLSPLYGRNHDEQMAVRTGKDGLLKPDTFSSKRVIGFPPGVGAFLIMFNRFHNYVVTQLAKINEGGRFKRPTTPDDTAGWETYDNSLFQTGRLITCGLYINIVLGDYVRTILNLNRANTTWNLDPRTKEGKSLLSKPTPEAVGNQVSVEFNLIYRWHCTISERDDKWTTNAMREALGGQDPATAKMEDVMRALGMFEKNIPDEPEKRTLAGLTRQSDGAFDDTELVKILQESIEDVAGAFGPNHVPACMRAIEILGIKQSRTWNVATLNEFRQFIGLTPHDSFYHMNPDPKICKILAQMYDSPDAVELYPGIMAEAAKPPFSPGSGLCPPYTTSRAILSDAVSLVRGDRFYTVDYTPRNITNWGFNEASTDKAVDWGHVIYKLFFRAFPNHFLPNSVYAHFPFVVPSENKLIFEGLGAANKYSWDPPKARAPIQFIRSHKAVLEVLSNQKDYKVTWGPAIKMLSGDPATSFALAGDEPANAASRHHVIAALTAPKQWRDEVRRFYEVTTRDLLRRHGAPVHGVGAGPRTHEVDVIRDVIGLAHARFMASLFSLPLKEEGKEEGAYGEHELYRSLVTIFAAIFWDSDVCNSLKLHQASKAAADKMSALIAEHVREMEAGTGFLGALGKLKDLITGNDVHANGNGVYTNGNGVYTNGNGVHTNGNGVHTNGNGVPHAAPSLRSFGDQLLQRMLSQDGRSIEETVSGTILPVVMAGTANQTQLLAQCLDYYLGVGEKHLPEMKRLAMLNTSEADEKLLKYTMEGCRIRGCVALYRAVVTDQAVDDTIPCIPNKDDPTFARPLSNPQVAESARTLKLSTGTRMLVDLTTASHDPAAFPDPDEVRLDRPLESYVHFGLGPHRCAGEPISQIALSSVMKVLLQLDGLRRAAGPRGEIRSYPASQWPGQAGRPPRDPAWSGLRTFTSADQSAFSPLATTMKINWEGRGDL

SEQ ID NO: 2 - protein, 773 aa, Nostoc sp.
MDLNTYLKLLNLLDSESQKIMLELQAMFSAAGLALRGRGTHTDGIIVKGNLTVLHSSDVPSHSLFTPGKKYDVIFRHANIVGGAKDDALINGRGSAIRIGNIGDDLSKPRLLDLVLNTGEVFGLPTARLYHQFFGSDFHQKSDMLASGSLRRYAVEAALRNPDSFTELYYHTQLCYEWVDSKKKSRYARFRLLNPNQSTEGGLLDDSVEIGPRLVLPRKRGDTREKNYLRNEFRQRLTDGNIVEYVLQAQFRSIEDVAVDCSNIWDPNTYPWLDIAAIVLNQDESENDYYQEIAYNPGNTHYDLKLPNSYSVDDFASLGVSGALVHYFGSIVRAERTQYLYGSKDDLPGKPVYFPLPVTEIPSKRFLFLLEKYNFLTDNSYPSDGEHDKIEALVSAMPTTALDLAVGTTDPTDIPDSYFLERRLNGYNPGAIRESSGQEGWTHELTHNLAKYDIKPGLHFPDFVQCRLFVDKQNGVKLHSIKIDDHEITPCQEQWQYAKRTYLQAEFLSQELKLHLARCHFNIEQYVMAIKRRLAPTHPVRAFINPHLEGLIFINSSAVPKIIGSTGFIPIASMLTQGSIVDVMKNELSKLSYMWNPIADLPRDIPGDLFTPAATAYWELLNNYVEQGLLQPFEDELRTEVNAIQVDELFAELKERSLYSGDQPPKYDSSELKSLLMYIIYHSSFLHSWANFKQYDDAGNPNHVSMGDYSQYDQQTQDKIRFSQRSLTWVLSSIRYNSVAVYGSDLLKQLIREKSSILEPGLPLEDLMMSINI

SEQ ID NO: 3 - protein, 805 aa, Acaryochloris marina
MDSRDPRTEHVDDEFKKLISNIARAFGRTAQIKGRRATHSYGTVAKGVLKVLDTLDIPQHQIFSAGKQYPVLLRHANIKGFRDDAILDGRGATVRVLAGDAQAPLSDLNLDEGIVDILMSTGRSFILAEALSFARWAAGPMKSRAAMLQEFPKIAPIFHEIIRDPDSYTQLHYYSETTYSFTSLNQQSFFLRYRLVNRQNPSADTGWLKPEEVKLPLDYLPRVASDTRPETYLQDDFRQQVRSTGVSYLLQIQLQPVSDDAAMNETAKDCTIPWEEEDHPFHDVAVLDLGSILPDELAEALEFNPYNAPPELSLILAKTARETASVNHLRSVVYQISANMRKYQTPSSSLVDWGSGHQPSLPEQYPYGTGKTPSFDNTKPLPARVKPKPRYWANFGLKLIPNQQLDPDLPELGITGALDLMGTSVVSYMPPNLTRTRLDKFSDDFFVERRLNGFNPGKLNRVTGHAWQYQVCYDCSKHQVEPAGILPTKITARFNFCGQYLHPHSIQFTLNGQTETQQPGDENWEWSKRLFRCAEFVFQEAQSHLGRTHMNLDQYAMAYYRNVVNNPIRLLLEPHLEGLLSINKLGANLISGPTGFIPEASSLTPESVDDVLKDEISHLSYHWTPHRQTLPDRVLNNHYDPAAIAMWNLLTQYVREFFEDHQAGMEEYWSEIQAMSHDLVTHSILKPELGTLAVQNNADLQQLCVYVIFLSSFFHSWVNNKQYEDGGDVSYSTIGLWDTRHPKYDPLRVAEREAKQVTLLWTLSHVRYNPIMDVGPTALKNLLWQQRQHIEPGIPLANLMMSTNI

SEQ ID NO: 4 - protein, 862 aa, Avena sativa
MLLGGLIDNLTGANKHARLKGTVVLMRKNVLDLNDFGATIIDGVSEFLGKGVTCQLISSTVVDNNNGNRGKVGAEAGLEQWLTSLPSLTTGESKFGLTFDWEVDKLGVPGAIVVNNYHSAQFFLKTITLDDVPGRAGKLTFVANSWIYPAEKYRYNRVFFANDTYLPSQMPAALKPYRDDELRNLRGDDQQGPYEEHDRVYRYDVYNDLGEDRPVLGGTADHPYPRRGRTGRKPNPNDPSLESRLSLLEQIYVPRDEKFGHLKMSDFLGYSIKAITQGILPAVRTYVDCTPGEFDSFQDIINLYEGGIKLPKIAALEELRKRFPFQLLKDLLPVGGDFLLKLPLPHIIKEDKQAWRTDEEFAREVLAGVNPVMITRLTEFPPKSTLDPSKYGDHTSTITAAHIEKNLEGLTVQQALEGNKLYILDHHDRFMPFLIDVNNLDGNFIYATRTLFFLRGDGRLTPLAIELSEPFIQDGLTTAKSKVYTPVPSGSVEGWVWELAKAYVAVGDSGWHQLVSHWLNTHAVMEPFVIATNRQLSVTHPVHKLLSPHYRDTMTINALARQTLINAGGIFEMTVFPGKFALGMSSVVYKDWNFAEQGLPDDLLRRGVAVPDPSSPYKVRLLIEDYPYAADGLAIWHAIEQYVTEYLAIYYPDDAVLQDDVELQAWWKEAREVGHGDLKDAPWWPSMQTVAELAKSCATIIWIASALHAAVNFGQYPYAGYLPNRPTVSRRRMPEPGTQEYAELERDPERAFIHTITSQIQTIIGISLLEVLSKHSSDELYLGQRDTPEWTSDPKALAVFQRFSDRLVDIESKVVGMNHDPQLKNRNGPAKLPYMLLYPNTSDRKGDAAGLTAKGIPNSISI

SEQ ID NO: 5 - protein, 863 aa, Oryza sativa [sequence omitted]

SEQ ID NO: 6 - protein, 619 aa, Magnaporthe oryzae
MRVLVWIAGLAPLAVAVPSSSYRVAVAARADNTSASVAPSQNVSGAAPPELVVYTLPCEDGNSTARTAEIRLKQATLLYGPSLLGNASYFPGGPLGDAISLRDQTVWEGAAVVQSLRAFTDAAKVAANIKQNGGLNSLDDFKVLYQDGWKGSVPQGIARGQSENYTSDLLFSMERLSVNPYILKRLHPTEDALPFQVDRATVKQLTKTSLKALHAAGRLFVADHSYQRNYTRLANRYSAACTALFYLDPRSNQFLPLAIKTNVGADLTYTPLDTDNNNWLLAKIMFNNNDLFHGQIFHVAYPHAIAEIVHLAALRTMSARHPVLALMERLMYQAYAVRPLGERVLFNKGGLFEQNFAYPQDMVYKFVGDSYPTTGRWRAGYLDTDVRARGLVDADYGPELPHFPFYEDGSRLVEVIRRFVRSFVDATYHESDEMVAKDAELQAWVAEANGPAGVEDFEPGPLDTRERLVEVLTHMAWLTGCAHHVLNQGEPVTASGVLPMHPTALYAPVPTSKANTTADLLGYLPSAQKSVDQVTLLARFNRPDVVPTNQTLRYMFAAPQLLLGNGEAYRRANQRFVRAMGRISDEVKARRFDDRGLSQGMPFIWQALDPGNIPFYLSV

SEQ ID NO: 7 - protein, 1121 aa, Aspergillus fumigatus
MLRRFSSTFKKKGDRESKQNGTASSSSAAVANTNNNDNKRHSKISAARKSSSDDDRNEKKGNSVSPFEKYASVLHASRSPIPNQTGDGAYLEHEHTTSLLQDARHLGFKDFKTLKEVIESKLPGGQLIDDKTMLMERIIQLVSRLPHNSKHREELTNAFLTELWDSLPHPPLSYMGNDYAYRSADGSNNNPTLPRLGAANTLYARTIPPLIIQPGGLPDPGLVFDTLFARQTFKPHPNKVSSVFFYWASLIIHDIFQTDYKNPNMNKTSGYLDLSILYGDVQEEQNLIRTFKDGKLKPDSFSEPRLQAFPATCCVLMVMLNRFHNYAVEQLAAINENGRFTKPADNLSEEEAKKAWAKYDEDLFQTGRLITCGLYINITLYDYLRTIVNLNRTNSTWCLDPRAQMEGSHTAPSGLGNQCSVEFNLAYRWHSATSATDEKWTEDVYERLMGKPASEVSMTELLMGLGKYQAELPKDPSKRTFADLERQADGRFKDEDLVNLLVNAVEDVAGSFGARNVPKVLKNVEILGIIQSRKWNVGSLNEFRKFFGLKPYETFEEINSDPDVAESLRSLYDHPDFVELYPGIVAEEAKQPMVPGVGIAPTYTISRAVLSDAVALVRGDRFYTIDYNPRNLTNWGYSEVRYDLSINQGCIFYKLATRAFPNWFKPDSIYAHYPMTIPSENRKIMKDLGREIHYSWDRPQYTPPRVDLVSYSNAKLVAEQQNQFRAAWGDTVEFVFGKASKEFKLYQDSAFIQKHADVMSKLLNKEEWHRSVKEFYEDITAKLLEDKTRRFGGINQVDITNDVGNLTPVIFAANVFSLPLKSKENPRGIYTEHEMFKVLAALYNCLYFDIDKTKSYPLHHASQAVGEPLGKALEANVKALGGSSLLSGIFRSFRENKNALKEYGVHLTKQLLENGLGAHEIAWAQFLPTVIAMVPAQAQAFTQIVDFYLSKEGSKHLPAIQRLAKQDTKKSDEQLLHYCLEAVRLNDMSGLYRQSETTLAVTDEAVEVTIQPGDKVFVSFAKANRDASVFPDPAEVRLDRPMNSYINPTLGPHGFLSKETSHIALTAMLRAVGRLNNLRVAPGVQGQLKKIPQPGGYSAYLREDHGSYSIFPTTFRVQYDA

SEQ ID NO: 8 - protein, 1117 aa, Aspergillus nidulans
MLRRFSTFRKSKGDKTEKADRDSKANGSNANSAAAASNSSKRQSKVPPPRRPSSDSGSSAESEDVPAVFEKYAQVLHASSRPIPHQGGEAAYLEKEHPSGLFNDLKSLGFKDFASLKDVIKTKINGELTDDKTMIMERIIQIVSSLPSNSKMRVDLTNMFLDELWGSLPHPPLSYMGNDYQYRSADGSNNNPTLPWLGAANTAYARSIEPLTVQPGGLPDAGLVFDTLFARQKFTPHPNKVSSLFFDWASLIIHDIFQTDYRDYNKNKTSAYLDLAILYGDVQEEQDLVRTHKDGKLKPDSFSEPRLQAFPAACCVLLVMLNRFHNYVVEELAAINENGRFTKPSPDLPEEQAKKAWAKYDEDLFQTGRLITCGLFINITLYDYLRTIVNLNRVNSTWCLDPRAQMEGSATPAGLGNQCSVEFNLAYRWHSAISANDEKWTEKVYEELIGKPGSEISTQELLMGLGKYGASLPKDPSQRTFAGLKRQEDGTFKDEELVNILTSAIEDVAGSFGARNVPKVLKAVEVLGIEQGRKWNVGSLNEFRKFFGLKNYETFEEINSDPEVAESLRALYGHPDYVELYPGIVSEEAKEPMIPGVGIAPTYTISRAVLSDAVALVRGDRHYTVDYNPRNLTNWGYNEVRYDLNINQGCVFYKLATRAFPNWFKPDSIYAHYPMTIPSENKVIMKNLGREADYSWDRPQYQAPRASLTSYSNVKLILDQQKDFRVVWGDCTPLHSGKGGEDFWSKTLSDPQFKKSIKEFYEKTTLELFADKSVNLAGRKQIDIVKDVGNIVPARFASKLLSLPLRSKENSKGVFTDHEIFMALAVIYNAIFFDVDTTKSFPLRKAADAVSKELGKHVESHVKSVSSPGFLSRVIDNFRDDHNALKDLGDQLIKRLAEGGLSVSDITYGQILPTAVELVHGQAQMFTRVVEYYLNEGKQHLPELSLLAKQDSAETDAKLTRYALEAIRLNAGSGAYRKAETNFYFKEGDADINLKPGDEIFISSTQANRDPTAFPDPDEVRLDRPDESYLNYGIGSQIGLGKDATLTAVTAMVRAAFSLEGLRPAPGVQGVLKKVVRPEGYTLYMREDHGAFSPFPTTFRVHFDGEVVTPKKQIDSA

SEQ ID NO: 9 - protein, 1113 aa, Aspergillus terreus
MLRRFSTQFKKSKGDRESKQNGTPGPANNSSKRQSKLAQPRKSSSSSSDGERSSKNEDGVPAFEKYAQVLHASRSPLPNQTGDGATSAHDHQTTLFQDLRSFGFKDFGTLKEVIATKAKGEHVDDKTMVMERIIQLVSGLPANSKSRTELTHLFLDQLWDSLPHPPLSYMGSDYAYRSADGSNNNPTLPWLGAANTPYARSIAPLTIQPGGLPDAGLVFDSLFARDKFRPHPNKVSSVFFDWASLIIHDIFQTDHQNPNINKTSGYLDLSILYGDVKEEQDLVRTHKDGKLKPDAFSEPRLQAFPATCCVLLVMLNRFHNHVVEQLAEINENGRFTKPSPDLPEDKAKAAWEKYDEDLFQTGRLITCGLYINITLYDYLRTIVNLNRVNSTWCLDPRAQMEGSSSTPSGLGNQCSVEFNLAYRWHSAISANDEKWTEQVYQDLMGKPAEEVSVEELLGGLMKYGRSLEKDPSKRTFAGLQRQADGTFKDEELVEILTNAVEDVAGSFGARHVPKALKAVEVLGINQARQWNVGSLNEFRKFFDLKPYESFEEINSDPDVADALRNLYEHPDYVELYPGIVAEEAKEPMIPGVGIAPTYTISRAVLSDAVALVRGDRHYTIDYNPRNLTNWGYNECRYDLSINQGCVFYKLATRAFPNWFKPDSIYAHYPMTIPSENRNIMKNLGRESHYSWERPKFTPPQVNLVSYPNVKLALEQEKQLRVIWSGNTPLRPAKGGDDFWSKALNNDEWRKNIKEFYEDMTIKLLNEKSCKLGGIRQIDITRDLGNLAPVHFASKVFSLPLKTKQNSKGVFTEHEMFMIMAVVFTSVFFDVDPTKSFPLHFASRAVSQQLGSAIESHVKSIGHPGFLSAIIDSFRDDDNVLKEYGDQLIKKLLDSGLGVSDVTYSQILPTAVSMVHNQARMFTHIVDYYVTEGKKHLPEINRLAKESTPEADEKLTRYCLEAFRLFGTFGSYREAQTDFTVNDESGPVDIKQGDKVFVGAVKANRDPSVFPDPDEVRLDRPLDSYIQFGLGPHAGLGKEATLLALTAMLRVVGRLDNLRPAPGPQGQLKKIPREGGYYVYLREDWGSYSPFPTTFKVHFDGELPAPKKRGIASA

SEQ ID NO: 10 - protein, 1117 aa, Aspergillus clavatus
MLRRFSSTFNKKKGDREPKQNGVATTTTTTTPTTNKRYSKVPEGHKSSSEEERNEKKGGAVSPFEKYASVLHASRTPIPNQTGDGAYLEHEHTTSLLQDARHLGFKDLATLKEVIKNKATGQLVDDKTMLMERVIQLVSSLPHNSKHREELTHSFLDELWGSLPHPPLSYMGSEYAYRSADGSNNNPTLPWLGAANTAYARTIAPLIIQPGGLPDPGLVFDTLFARQSFKPHPNNVSSLFFDWASLIIHDIFQTDYRNPHVNKTSGYLDLSILYGDVQEEQNLIRTFEGGRLKTDSFSEPRLQAFPAACCVLLVMLNRFHNHVVEQLAAINENGRFTQPRDGLPEDQAKKAWEKYDEDLFQTGRLITCGLYINITLYDYLRTIVNLNRTNSTWCLDPRAQMEGNNTTPSGLGNQCSVEFNLAYRWHSAISANDEKWTEKIYEDLMGKPASEVSMTELLMGLGKYEAGLSKDPSQRTFAGLERQADGRFRDEDLVNILTGAIEDVAGSFGARNVPKVLKNVEVLGILQSRKWNVGSLNEFRKFFGLKPYETFEEINSDPDVAESLRSLYDHPDFVELYPGIVSEEAKEPMIPGVGIAPTYTISRAVLSDAVALVRGDRYYTIDYNARNLTNWGYSEVRYDLSINQGCVFYKLATRAFPDWFKSDSIYAHYPMTIPSENRKIMKNLGREAHYSYDRPQYIPPPVDLLSYPSAKLVAEQRKDFHTVWADTVEFVFGKASKNFKLSEDTAFIERQRETISKLLSQDEWQRNVKEFYEEITTGLLEEKTRRFAGINQVDITRDIGNLVPVIFASNLFSLPLRSKENSRGIFTEHEMFNVLAVLYNCIYFDIDKTKSFPLHHASQAVGEQLGKAVEANVKSLGGSSLLSGILGGSRDNKNALKEYGAHMTKQLLENGLGASEITWSQILPTVIAMVPSQAQAFTQIIDFYLSKEGSKYLPEIQRLAREESKESDEQLLRYCMEAIRLNKTSGAYREARTSLTVTEETGQVTLQPGDKVFVGFAKANRDPSVFPDPSEVRLDRPLDAYINHSLGPHGFLSKETSQIALTAMLRAVGRLNNLRRAPGAQGEVKKVPIADGYSAYLREDHGSYSVFPTTFRVHYDV

SEQ ID NO: 11 - protein, 1125 aa, Penicillium marneffei
MRRFSSVFKKKEESKAKENGHISEKVNGKRQSKAVSTSQPPAEPEDHSKARHEVSAIFERYAQVIHASRQPLPTQSGDGTYLEHGHDHSSSLFSDLRSLGFKDYGTLVEVMKNKASGSYVDDKTMLMERIIQLVSGLPSNSERRTELTNAFLDELWDSLPHPPLSFVGPKFEYRSADGSWNNPTIPWLGAANTEYSRSIPPLTIQPSGLPDAGLVFDSIMAREKFTPHPNKVSSVFFAWASLIIHDIFQTDYRNPHISQTSSYLDLSILYGDNQDDQNQMRTFKDGKIKPDSFSEPRLQAFPAMCNVLMVMLNRFHNNVVEQIAQINENGRFNKPRPGLSPEQTEAAWKKYDEDLFQTGRLITCGLYINITLYDYLRTIVNLNRTNSTWCLDPRARMQGTHTTPSGLGNQCSVEFNLAYRWHSATSYNDEKWTEEVYRDLFGKPAEEISMPELLMGLHKYEQSIDKDPSKRTFANLQRQADGTFKDDDLVKIMTSAVEDVAGSFGARNVPKVMRSIEILGIEQARKWNVGSLNEFRKFFNLKPYETFEEINSDPYVADQLRHLYEHPDYVELYPGIVAEEAKAPMVPGVGIAPTYTISRAVLSDAVALVRGDRFYTTDQTPRNLTNWGWQESGHDLNINQGCVFYKLAFRAFPNHFKPDSIYAHYPMTIPEENKVIMKDLGREDDYSWDQPTFNAPRVELKTYQAAQTVLNDTRNFRVTWGDASAWVFGEKTGFDYMLSGDTPFHGQQRELLERSLYQEGWDSRLKEFYEQITLQLLHDKSYTLAGTKQVDLTRDVGNLATVHFAAHLFGLPLKTKGNPRGIFTEHELYMANAVIFQAVFFDYDLMRSYPLRQAARAVAKKIGEMVELNVKSIGSNGIISHFIDGLRKQDNPLSDYGENLVKKLLDSGLNAHEVTWTQILPAVVSMVPKLGQVFTQIIDFYLSDAGKAYLPEINRLTKLNTPESDQALTHYVLEAIRLNGTYGAYREAQRDVTVNDGGNEIQVNKGAKVFVSFISASRDPAAFPEPEKVVLDRPVESYVHYGIGPHSCLGQDASLIALTSMLRVVGRLENLRRARGTQGLLKKIPREGGSYHYLREDGGSFTPFPATFKVEWDSELPPLKNRGTW

SEQ ID NO: 12 - protein, 1117 aa, Penicillium decumbens
MLRRFSTQFRKNKESNSDADSSKNSKENGKRHSKPIQPSRKASSHDEKQHSVNRAEVVAVFEKHAQAIHASREPLPSQGGDGAYLKHDQSSGLFEDIKSLGFRDLSTVKSLIKSKASGELIDDKTYLMERIIQLVADMPGHSKNRVELTNQFLDELWDSLPHPPLSYMGDEYKYRSADGSRNNPTLPQLGAANTPYCRTIPPLTIQPSGLPDAGLLFDSLFARQKFTPHPNKVSSIFFDWASLIIHDIFQTDYRQQHVNKTSSYLDLSILYGDVKEQQDLIRSHQDGKLKPDCFSEGRLQALPAACGVLLVMLNRFHNHVVEQLAAINENGRFTKPLDGLPEDAAKKAWAKYDEDLFQTGRLITCGLYINITLYDYLRTIVNLNRTNSTWCLDPRAQMEKTGATPSGLGNQCSVEFNLAYRWHSTIAQGDEKWIEQIYYDLMGKPAEEVSMHELLMGMKKVEGSLDPDPSKRTFARLERQADGTFKDEELVAILTSACEDVASSFGPRNVPKALRSIEILGIEAARRWHVGSLNEFRKHFGLKPYDTFEEINSNPEIANCLRHLYEHPDYVELYPGIVSEEPKEPMVPGVGIAPTYTISRAILSDAVALVRGDRHYTIDYNARNLTNWGYNECRYDLNINQGCVFYKLALRAFPNWYKPDSIYAHYPMTIPSENRNIMKSLGREQDYSWERPSFTPSRINLSSHNNARLVLENSTDFTPVWSEAMTELFGKGEFGAQQREAMSAAFATEDFLTLVKNFYEEVTLRLIKEKGANLVGTNQVDITRDVGNLAHVHFASALFGLPLKTDENPRGLFTEHEMYMILATIYSALFYDVDPAKSLPLNSAASAVARQLGSVVEATVKTDTHSGLFSGLINSFRPHDNAIREHGTAALRRVEESGQSASQITWSHIIPTVVGMVPSQGQVFTQVIEYYTSPEGKHHWSEISRLARQDSKESDEMLHRYCLEAIRINGTFGEYREAKNPVILEENEEVINVQPGNKIFASFIQANLDPSVFPEPNSVNLSRPLSSYIHQGQGPANGLGQETTKIALVSMLRVVARLPNLRRAPGAQGQLKRIPQKGGHYVYLRQDGTSYFPFPTTLKLHWDGDFEFQTSQTSKKH

SEQ ID NO: 13 - protein, 1118 aa, Penicillium chrysogenum
MLKRFSTQFKRSKDSKDPKESNGDAEPKSTDKSSKRASKVSPSPKSTHKEENHVVKRSEVVAVFDKYAQAIHASQEPLPNQTSDGAYLKHDKSSGLINDIKALGFRDVGTVKDLIASKASGGIIDDKTYLMERIIQMVADLPGNSKNRTDLTGLFLDDLWNSIPHPPLSYMGDDYKYRSADGSNNNPTLPWLGAANTPYCRTIAPLTIQPSGLPDAGLIFDTLYARQEFTPHPNKVSSVFFDWASLIIHDIFQTDYSQQHLNQTSAYLDLSILYGDVKEQQDKIRSHENGKLKPDCFSEGRLQALPPACGVLLVMLNRFHNHIVTQLAAINENGRFSAPRPGLSEEETKAAWAKRDEDLFQTGRLITCGLYINITLYDYLRTIVNLNRTNSTWCLDPRAQAEKADATPSGLGNQCSVEFNLAYRWHSTISQGDEKWIEQIYYDLMGKPAEQVSMPELLMGMKKVKGMLEADPAKRTFGHLQRNADGYFDDGELVNILTRATEDVASSFGPRNVPKAMRSIEILGIEASRRWNVGSLNEFRKHFGLKPYETFEDVNSNPEIANTLRHLYEHPDYIELYPGIVSEEAKEPMIPGVGIAPTYTISRAVLSDAVALVRGDRHYTIDYNPRNLTNWGYNECRYDLNINQGCIFYKLATRAFPNHYKPDSIYAHYPMTIPSENRNIMKDLGREQDYSWDKPAFMEPRVNLTSHQNAKLLLENQKDFRPSWARSMSELFGKGEFDTKQREAIGKALNTEEFPKLVKTFYEDITERLIAEKGGQLGKINQIDITRDVGNLAHVHFASTIFGVPLKTEDNPRGLFTEHEMYMILSTIFSALFFDVDAPRSYALNRAASAVSNQLGQVVEATVKADTNSGLFAGIMDNFRPHDNALREFGTEAIRRMKEAGSSASDITWSAIVPTIVGLVPNQAQVFTQIIEFYTAPENKAHLAEINRFAKTDSAESDEKLYRYCLEAVRLNGTFGAFREAKETVTVEEDGKTYTVQPGQQVFASFDQANHDPSVFPEPNEVNLDRPLDSYINHGQGPTTGFGEQVTKIALIAMLRVVGRLQGLRRAPGAQGQLKKIPQEGGYQVYLRGDGTAYCPFPMSLKLHWDGPFEQKKKVTSS

SEQ ID NO: 14 - protein, 1110 aa, Aspergillus niger
MLRRFSSTFKRSSKGDRDSKPNGTQVNGQKRQSKVPAPRKSSSDESHSDHGVESDDGVSVFEKYAQVLHASRRPLPNQNGDGTYLEQEHSGSLFKDLRALGFKDIGTLKDLIKTKAKGEYIDDKTMLMERIIQLVSSLPGNSKTRVDLTNAFLDELWGSLPHPPLSYMGEEYAYRSADGSNNNPTLPWLGAAGTPYARSIAPLTIQPGGLPDAGLVFDCLFAREKFTPHPNKVSSLFFDWASLVIHDIFQTDYTNSHVNKTSAYLDLSILYGDDQEDQNLVRTFKDGKLKPDTFSEQRLQAFPPACSVLMVMLSRFHNWVVEELAAINENGRFNKPDPRLDEEKARKAWEKYDNDLFQTGRLVTCGLFINITLYDYLRTIVNLNRSNSTWCLDPRVQMEGTKSTPSGLGNQCSVEFNLAYRWHSAISANDEKWTEEIYEELMGKPASEVSMRELLVGLGKYEREIPKDPSKRTFAGLKRQEDGTFKDEDLVRILANAIEDVASSFGARNVPKVLRSVEILGIEQGRKWNVGSLNEFRKFFDLKPYETFEEINSDPDVADSLRHLYEHPDYVELYPGIVAEEAKEPMIPGVGIAPTYTISRAVLSDAVALVRGDRYYTIDYNPRNLTNWGYNEVRYDLNINQGCVFYKLAMRAFPNYFKPDSIYAHYPMTIPSENRNIMKNLGRESHYSYDRPRYTEPVPNLLSYANAKLVLNNQKDFTVPWGGLSSIHAGKGGADFWSKSFDNEQWRNSVKEFYEDATLKLLNEKSCKLAGNKQVDIARDVGNLVPVHFVSKVFSLPLKTKSNPRGIFTEHEMFMIMAVVFNSTFFDVDPTKSFPLQHAARAVSQELGKVVEAHVKSINHPGFLHGIIDSFRDDHNALKDYGDQLIKRLLESGLGVSDVTWGQILPAAVEMVHTQSQMFTQIIHFYLTEGQKYLPEINRLANENTAEANDRLTRFCLEAVRLNGNLGIYREAQADINVSDETGQYSVKSGEKVFVGSSKANRDPQAFPSPDEVRLDRPLDSYLHYGLGPQSGLGKDATLAAVTAMVRVVARLDTLRPAPGAQGQLKKIPQEAGFSVYMREDYGSYSPFPTTYKVHYNGDVPAPKRQVTTA

SEQ ID NO: 15 - protein, 542 aa, Nostoc punctiforme
MAGKRDTSKDGLGNKIQTLVLTNFKGLWQLLQSNEFIKRKVNKTLLNSLIYKIPTRPNAYSMMTLDEHIPDTNIPKKTDTYTSWESLNDRTYTGRHLPPDPKLNAEGNLPKVEDLAILFRKRDGKTIYSGKSTMLFPYWVQWFTDSFLRLNHYNKLKNTSNHEIDLCNVYGLTRKQTHLLRSFQGGKLKTQKLKRQDGVEEEYPLFYYADPAQDKVKPEFEGLYEPINDEKRQPIDKKQYMFAMGVERANVQIGYVMLNTLCFREHNRLCDELARNYPDWDDERLFQTSRNILMAIILKIIMEEYINHITPYHFKLFADPEAFTKESWHRPNYMAIEFDFVYRWHSAIPETFNYNGKPTHIVTSLWNNKMFIDQGLGALMEETCSQPGTKIGLFNTPDILVELTELPSIRLGRQLQLASYNDYRELCGFPRVTRFEQVTGNEFAQEKLKELYGHVDKIEFFVGLYAEDGRENSTIPALVARLIGIDAFSQALTNPLLSPNIFNKETFSPVGWEILQNTKTVSDLVNRNVPPSGKKYKVTFDL

SEQ ID NO: 16 - protein, 634 aa, Pseudomonas aeruginosa
MTLSRLSLAILSVLAGAPAFADDSGVDLDQGWNQTQKTAWLEAGQGSRMLPLAWLVALEQRASEEPLMSDALIRQYGYVPHTLGGSSVKVVQGYAVDRSDDSDLTFTKLRWKALQGSREPWVGPTCSMCHTSHISYQGTQLTVYGGQTMGDLAGFQLEILGALQSTRADTAKFERFARKVLGADGLVSGYNDANKARLQAALDATIVRLRDGSHFNLPHDPEFGPGRLDAIGSIFNSVGYELHADEQIYGAEDAPVSYPFLWNVPQLDRVQWTGFNPNHINVVDIDNRKFDVGALARNAGEAVGVFADVKVLSPIQSALHIGYPSSINVDNLIRIEDQLGQLKPPAWPNQLFGAPEPTRVAEGRELYRQHCSSCHTPLDRNDLRTPVKTVLTHLQARGEVAPIGTDPWTACNSIAQLKTGYVRGKPYLSFVGTGQRGFYGKQAYAVDVLQEVVVQALAARGLSVALGAFQTAALGIFDGQLPPLISPVPDSPDADSAEATAADAPGALLLAENVAADSDKARRLEQCLAMTSDLMAYKARPLNGIWASPPYLHNGSVATLYDLLLPPDLRPRTFYTGSVEFDPVNVGYITDAGGANRFLFDSGKPGNANGGHDYGNAQFNEQQRRALVEYMKTL

SEQ ID NO: 17 - protein, 634 aa, Pseudomonas aeruginosa
MTLSRLSLAILSVLAGAPAFADDSGVDLDQGWNQTQKTAWLEAGQGSRMLPLAWLVALEQRASEEPLMSDALIRQYGYVPHTLGGSSVKVVQGYAVDRSDDSDLTFTKLRWKALQGSREPWVGPTCSMCHTSHISYQGTQLTVYGGQTMGDLAGFQLEILGALQSTRADTAKFERFARKVLGADGLVSGYNDANKARLQAALDATIVRLRDGSHFNLPHDPEFGPGRLDAIGSIFNSVGYELHADEQIYGAEDAPVSYPFLWNVPQLDRVQWTGFNPNHINVVDIDNRKFDVGALARNAGEAVGVFADVKVLSPIQSALHIGYPSSIKVDNLIRIEDQFGQLKPPAWPNQLFGAPEPTRVAEGRELYRQHCSSCHTPLDRNDLRTPVKTVLTHLQARGEVAPIGTDPWTACNSIAQLKTGYVRGKPYLSFVGTGQRGFYGKQAYAVDVLQEVVVQALAARGLSVALGAFQTAALGIFDGQLPPLISPVPDSPDADSVEATAADAPGALLLAENVAADSDKARRLEQCLAMTSDLMAYKARPLNGIWASPPYLHNGSVATLYDLLLPPDLRPRTFYTGSVEFDPVNVGYITDAGGANRFLFDSGKPGNANGGHDYGNAQFNEQQRRALVEYMKTL

SEQ ID NO: 18 - protein, 610 aa, Fusarium oxysporum
MVALLIFLGIFTCVETLPLSDSPSSYIPEEVPSSQTADIGLPPPTEFTLPNEDDEILIRKLNIQKTRKEILYGPSLIGKTSFFISGPLGDQISQRDQTLWSRDAAPVVQAVSHDAAAALHDIQIHGGLQNLDDYKILYQGHWSSSVPGGIAKGQFSNFTSDLLFSMERLSTNPYILRRLHPHADELPFAVDSKIVQKLTGSTLPSLHKAGRLFLADHSYQKDYVAQEGRYAAACQALFYLDDRCHQFLPLAIKTNVGSNLTYTPLDEPNDWLLAKVMFNVNDLFHGQMYHLASTHAVAEIVHLAALRTMSSRHPVLALLQRLMYQAYAIRPIGNNILFNPGGLIDQNSVFSNVAVRKFATDFYPTVAGPVRSNYFEANLRSRGLLNATHGPDLPHFPFYEDGARIIKVIRTFIQSFVKSIYKSDKVLAKDWELQAWIAEANGAAEVIDFPPTPLKKRKHLVDILTHMAWLTGVSHHVLNQGEPVTTSGVLPLHPGSLYAPVPGEKGVVDSLLPWLPNEQKSVDQISFLALFNRPQIVENNRTLRYMFNSESLLAGTVRAVAAANERFMEEMGHISQEISNRKFDDDGLSQGMPFIWTGMDPGVIPFYLSV

SEQ ID NO: 19 - protein, 618 aa, Gaeumannomyces graminis
MRSRILAIVFAARHVAALPLAAEDAAATLSLTSSASSTTVLPSPTQYTLPNNDPNQGARNASIARKRELFLYGPSTLGQTTFYPTGELGNNISARDVLLWRQDAANQTATAYREANETFADITSRGGFKTLDDFALLYNGHWKESVPEGISKGMLSNCTSDLLFSMERLSSNPYVLKRLHPTKDKLPFSVESKVVKKLTATTLEALHKGGRLFLVDHSYQKKYTPQPGRYAAACQGLFYLDARSNQFLPLAIKTNVGVDLTYTPLDDKDDWLLAKIMFNNNDLFYSQMYHVLFHTIPEIVHEAAFRTLSDRHPVMGVLNRLMYQAYAIRPVGGAVLFNPGGFWDQNFGLPASAAIDFPGSVYAQGGGGFQAGYLEKDLRSRGLIGEDSGPRLPHFPFYEDAHRLIGAIRRFMQAFVDSTYGADDGDDGALLRDYELQNWIAEANGPAQVRDFPAAPLRRRAQLVDVLTHVAWITGGAHHVMNQGSPVKFSGVLPLHPAALYAPIPTAKGATGNGTRAGLLAWLPNERQAVEQVSLLARFNRAQVGDRKQTVRDAFAAPDLLAGNGPGYAAANARFVEDTGRISREIAGRGFDGKGLSQGMPFVWTALNPAVNPFFLSV

SEQ ID NO: 20 - protein, 609 aa, Colletotrichum gloeosporioides
MRLLLSIAGLTTVVNALAVRADGNVTSSTAVATPTAWTGFPVPTEYTLPQDDHDFQERKEEIKLKRDTITYVPSIIGETSLFIGGSVGTQIVRQEQAKWIQDLTPVQQDAFREGNASLKAIQDHGGLKTLEDYKILYDGHWSGSVPGGIAQGQFNNFTSDLLFAMERLSTNPYVVRRLNPESDKIPFSVDANNVTHLTGTTLDTLFKSGSLFLADHSYQAEYTAQDGRYSAACQALFFLDQRSGQFLPLAIKTNVGSDLVYTPLDDPNDWLLAKIMYNVNDFFHGQIYHLANSHAVAEIVNLAAIRTLSSRHPVFGLLQRLMFQAYAIRATGEIALFNPGGLFDQSFAFSNVYARKFATDFYPTVAGPFQANYFEEDLRARGLLNASYGPELPHLPFHEDGHKIINAIRTFIGTFVDTVYESDKVLAEDSELQAWIAEANGPAKVINFPSAPLNTRKQLAEILTHMAWLTGVSHHVLNQGEPFTTSGVLPLHPASLYAPVPTAKGGIKDLLPWLPNEQKSVEQISLLARFNRPKIVENNETLLHMFDVKTLLSGTGEAVKAANEQFMIAMGTISKEISTRKFDDQGLSQGMPFIWTGMDPGVIPFYLSV

SEQ ID NO: 21 - protein, 896 aa, Arabidopsis thaliana
MYCRESLSSLQTLNVAKSLSSLFPKQSALINPISAGRRNNLPRPNLRRRCKVTASRANIEQEGNTVKEPIQNIKVKGYITAQEEFLEGITWSRGLDDIADIRGRSLLVELISAKTDQRITVEDYAQRVWAEAPDEKYECEFEMPEDFGPVGAIKIQNQYHRQLFLKGVELKLPGGSITFTCESWVAPKSVDPTKRIFFSDKSYLPSQTPEPLKKYRKEELETLQGKNREEVGEFTKFERIYDYDVYNDVGDPDNDPELARPVIGGLTHPYPRRCKTGRKPCETDPSSEQRYGGEFYVPRDEEFSTAKGTSFTGKAVLAALPSIFPQIESVLLSPQEPFPHFKAIQNLFEEGIQLPKDAGLLPLLPRIIKALGEAQDDILQFDAPVLINRDRFSWLRDDEFARQTLAGLNPYSIQLVEEWPLISKLDPAVYGDPTSLITWEIVEREVKGNMTVDEALKNKRLFVLDYHDLLLPYVNKVRELNNTTLYASRTLFFLSDDSTLRPVAIELTCPPNINKPQWKQVFTPGYDATSCWLWNLAKTHAISHDAGYHQLISHWLRTHACTEPYIIAANRQLSAMHPIYRLLHPHFRYTMEINARARQSLVNGGGIIETCFWPGKYALELSSAVYGKLWRFDQEGLPADLIKRGLAEEDKTAEHGVRLTIPDYPFANDGLILWDAIKEWVTDYVKHYYPDEELITSDEELQGWWSEVRNIGHGDKKDEPWWPVLKTQDDLIGVVTTIAWVTSGHHAAVNFGQYGYGGYFPNRPTTTRIRMPTEDPTDEALKEFYESPEKVLLKTYPSQKQATLVMVTLDLLSTHSPDEEYIGEQQEASWANEPVINAAFERFKGKLQYLEGVIDERNVNITLKNRAGAGVVKYELLKPTSEHGVTGMGVPYSISI

SEQ ID NO: 22 - protein, 941 aa, Oryza sativa
MLRPQLNPSSSHHHTTTTSSSSSTQLYFASSSCIASLRRPSPPSLIAGAGCRTTRRRQQGRQRVVVRCASSSAASSASEAARRGTGSSDMAPAAVVKVKAVATIKVTVEGLLNSLRPSKAIDNIRDLIGRSLFLELVSSELEAKTGKKKATVHSYAHKVDDDDHGVVTYEADFDVPTGFGPIGAVVVTNELGQEMFLEDLNLTAGDGAGNSTVLPIRCNSWVQPKSSIDEGTPGKRIFFAKAYLPGQTPAGLRSYREEDLKQKRGNGAGQREADDRVYDYDVYNDLGNPDSNGDLARPVLGGSKQFPYPRRCRTGRPPSKKDPKSETRKGNVYVPRDEEFSEVKNAQFLLKTLQSVLHAAVPAAQSALIDNLSLNLPFPSFFVIDKLFEDGVELPGVEKLGFLHSIVPRLLELLRDSPGDKILLFDTPANVQKDKFAWLRDEEFARETLAGINPYAIELVREFPLKSKLDPAVYGPAESAITADLLEEQMRRVMTVEEAISQKRLFMLDFHDLFLPYVHKIRSLKHTTMYGSRTIFFLTDDGTLRLLAIELTRPASPSQPQWRQVFTPSTDTTKSWLWRMAKAHVRAHDAGHHELITHWLRTHCAVEPYIIAANRQLSEMHPIYQLLHPHFRYTMRINALARSRLISAAGIIELSFSPQKYSMELSSVAYDKLWRFDMEALPADLVRRGMAEEDPTAEHGLRLAIEDYPFANDGLLIWDAIKTWVQAYVARFYPDADSVAGDEELQAFWTEVRTKGHGDKKDAPWWPKLDSPESLAHTLTTIVWVAAAHHAAVNFGQYDFGGYFPNRPSIARTVMPVEEPVDGAAMERFLDNPDQALRECFPSQVQATVVMAVLDVLSTHSTDEEYLGGEQTRPWNSDAAVQAAYAGFTARLKEIEGVIDGRNKDRKLKNRCGAGILPYQLMKPFSDAGVTGMGIPNSTSI

SEQ ID NO: 23 - protein, 685 aa, Pseudomonas aeruginosa
MKRRSVLLSGVALSGTALANDSIFFSPLKYLGAEQQRSIDASRSLLDNLIPPSLPQYDNLAGKLARRAVLTSKKLVYVWTENFANVKGVPMARSVPLGELPNVDWLLKTAGVIVELIVNFVASLPASAAAQFERIAAGLSGDLEAARQVHEALLEEAKNDPAAAGSLLLRFTELQTRVIALLTRVGLLVDDILKSASNLVTQGGQGDGLNRFRAVFGTLRLPEVADSFRDDEAFAYWRVAGPNPLLIRRVDALPANFPLGEEQFRRVMGADDSLLEAAASRRLYLLDYAELGKLAPSGAVDKLLTGTGFAYAPIALFALGKDRAGLLPVAIQCGQDPATHPMFVRPAESESDLYWGWQMAKTVVQVAEENYHEMFVHLAQTHLVSEAFCLATQRTLAPSHPLHVLLAPHFEGTLFINEGAARILLPSAGFIDVMFAAPIQDTQATAGGNRLGFDFYRGMLPESLKARNVDDPAALPDYPYRDDGLLVWNAIRQWAADYVAVYYASDGDVTADVELAAWVGEVIGSGKVAGFRPITGRSQLVEVLTMVIFTASAQHAAVNFPQPSMMTYAPAICAMSAAPAPDSPSGKSEADWLKMMPPTLVALEKVNIYHLLGSVYHGRLGDYRQTGFPYAPVFSDRRVTASGGPLERFQARLKEVEATIRTRNQARRKPYEYLLPSRIPASTNI

SEQ ID NO: 24 - protein, 880 aa, Momordica charantia
MFGIGKSIIEGAVNTTGDLAGSVINAGGNIVGRVTNIGGKKIKGTVVLMRSNVLDFTEFHSSLLDGVTELLGGGISLQLISATHASNDSRGKVGKGAFLERWLTSVPPLFAGESVFQVNFDWEENFGFPGAFFIKNGHTSEFFLKSVTLEDVPGFGRVHFDCNSWVYPSRRYKKDRIFFANHTCLPIDTPDSLRKYREEELLNLRGDGTGERKEWDRIYDYDVYNDLCDPNGGPNLVRPILGGSDQYPYPRRGRTGRPPARKDHKYESRLSDVMSLNIYVPRDENFGHLKMADFLGNTLKVLSTSIQPGLESIFDSTPGEFDKFKEVDDLFERGFPIPLNIFKNLTEDLAPPLFKAFLRSDGERFLKYPTPQVIKDNKLGWRTDEEFAREMIAGVNPLIIRRLEVFPPLSKLDPHVYGNQNSTMTEEQIKHGLDGLTVDEAIKENKLYILDHHDALMPYLRRINSTSTKTYATRTLLFLKDDSTLKPLAIELSLPHPQGDEHGAISKLYFPAEGRVESAIWQLAKAYVAVNDSGYHQLNSHWLHTHAVLEPFVITTHRRLSVLHPIHKLLAPHYKDTMFINASARQVLINAGGLIESTQFPAKYAMELSSYIYKEWKFPDEALPTNLIKRGVAIEDSGSPHGVRLLINDYPFAVDGLEIWSAIKTWVTDYCSLYYKDDDAIRNDVELQSWWKELREKGHTDKKDEPWWPKMQTFSELIESCTIIIWISSALHAAVNFGQYPYGGYVPNRPTTSRRFMPEVGTAEYKEVESNPEKAFLRTISSQIVALLGLSIIEILSKHASDEVYLGQRASIEWTSDKSAIEAFEKFGKELFEVEDRIMRRNQDVNLKNRAGPVNMPYTLLVPSSTEGLTGRGIPNSISI

SEQ ID NO: 25 - protein, 674 aa, Homo sapiens
MPSYTVTVATGSQWFAGTDDYIYLSLVGSAGCSEKHLLDKPFYNDFERGAVDSYDVTVDEELGEIQLVRIEKRKYWLNDDWYLKYITLKTPHGDYIEFPCYRWITGDVEVVLRDGRAKLARDDQIHILKQHRRKELETRQKQYRWMEWNPGFPLSIDAKCHKDLPRDIQFDSEKGVDFVLNYSKAMENLFINRFMHMFQSSWNDFADFEKIFVKISNTISERVMNHWQEDLMFGYQFLNGCNPVLIRRCTELPEKLPVTTEMVECSLERQLSLEQEVQQGNIFIVDFELLDGIDANKTDPCTLQFLAAPICLLYKNLANKIVPIAIQLNQIPGDENPIFLPSDAKYDWLLAKIWVRSSDFHVHQTITHLLRTHLVSEVFGIAMYRQLPAVHPIFKLLVAHVRFTIAINTKAREQLICECGLFDKANATGGGGHVQMVQRAMKDLTYASLCFPEAIKARGMESKEDIPYYFYRDDGLLVWEAIRTFTAEVVDIYYEGDQVVEEDPELQDFVNDVYVYGMRGRKSSGFPKSVKSREQLSEYLTVVIFTASAQHAAVNFGQYDWCSWIPNAPPTMRAPPPTAKGVVTIEQIVDTLPDRGRSCWHLGAVWALSQFQENELFLGMYPEEHFIEKPVKEAMARFRKNLEAIVSVIAERNKKKQLPYYYLSPDRIPNSVAI

SEQ ID NO: 26 - protein, 1066 aa, Plexaura homomalla
MTWKNFGFEIFGEKYGQEELEKRIKDEHTPPPDSPVFGGLKLKLKKEKFKTLFTLGTTLKGFRRATHTVGTGGIGEITIVNDPKFPEHEFFTAGRTFPARLRHANLKYPDDAGADARSFSIKFADSDSDGPLDIVMNTGEANIFWNSPSLEDFVPVEEGDAAEEYVYKNPYYYYNLVEALRRAPDTFAHLYYYSQVTMPFKAKDGKVRYCRYRALPGDVDIKEEDESGRLTEEEQRKIWIFSRHENEKRPDDYLRKEYVERLQKGPVNYRLQIQIHEASPDDTATIFHAGILWDKETHPWFDLAKVSIKTPLSPDVLEKTAFNIANQPASLGLLEAKSPEDYNSIGELRVAVYTWVQHLRKLKIGSLVPAGQNAIYNVEVETGDREHAGTDATITIRITGAKGRTDYLKLDKWFHNDFEAGSKEQYTVQGFDVGDIQLIELHSDGGGYWSGDPDWFVNRVIIISSTQDRVYSFPCFRWVIKDMVLFPGEATLPFNEVPAIVSEQRQKELEQRKLTYQWDYVSDDMPGNIKAKTHDDLPRDVQFTDEKSRSYQESRKAALVNLGIGSLFTMFENWDSYDDYHILYRNWILGGTPNMADRWHEDRWFGYQFLNGANPVILTRCDALPSNFPVTNEHVNASLDRGKNLDEEIKDGHIYIVDFKVLVGAKSYGGPVLEDIGYKVPDHLKHDEADIRYCAAPLALFYVNKLGHLMPIAIQINQEPGPENPIWTPHEENEHDWMMAKFWLGVAESNFHQLNTHLLRTHLTTESFALSTWRNLASAHPVFKLLQPHIYGVLAIDTIGRKELIGSGGIVDQSLSLGGGGHVTFMEKCFKEVNLQDYHLPNALKKRGVDDPSKLPGFYYRDDGLALWEAIETFIGEIIAIFYKNDDDVKRDNEIQSWIYDVHKNGWRVNPGHQDHGVPASFESREQLKEVLTSLVFTFSCQHAAVNFSQKDHYGFTPNAPAVLRHPPPKKKGEATLQSILSTLPSKSQAAKAIATVYILTKFSEDERYLGNYSATAWEDKDALDAINRFQDKLEDISKKIKQRNENLEVPYIYLLPERIPNGTAI

SEQ ID NO: 27 - protein, 663 aa, Homo sapiens
MGRYRIRVATGAWLFSGSYNRVQLWLVGTRGEAELELQLRPARGEEEEFDHDVAEDLGLLQFVRLRKHHWLVDDAWFCDRITVQGPGACAEVAFPCYRWVQGEDILSLPEGTARLPGDNALDMFQKHREKELKDRQQIYCWATWKEGLPLTIAADRKDDLPPNMRFHEEKRLDFEWTLKAGALEMALKRVYTLLSSWNCLEDFDQIFWGQKSALAEKVRQCWQDDELFSYQFLNGANPMLLRRSTSLPSRLVLPSGMEELQAQLEKELQNGSLFEADFILLDGIPANVIRGEKQYLAAPLVMLKMEPNGKLQPMVIQIQPPNPSSPTPTLFLPSDPPLAWLLAKSWVRNSDFQLHEIQYHLLNTHLVAEVIAVATMRCLPGLHPIFKFLIPHIRYTMEINTRARTQLISDGGIFDKAVSTGGGGHVQLLRRAAAQLTYCSLCPPDDLADRGLLGLPGALYAHDALRLWEIIARYVEGIVHLFYQRDDIVKGDPELQAWCREITEVGLCQAQDRGFPVSFQSQSQLCHFLTMCVFTCTAQHAAINQGQLDWYAWVPNAPCTMRMPPPTTKEDVTMATVMGSLPDVRQACLQMAISWHLSRRQPDMVPLGHHKEKYFSGPKPKAVLNQFRTDLEKLEKEITARNEQLDWPYEYLKPSCIENSVTI

SEQ ID NO: 28 - protein, 701 aa, Homo sapiens
MATYKVRVATGTDLLSGTRDSISLTIVGTQGESHKQLLNHFGRDFATGAVGQYTVQCPQDLGELIIIRLHKERYAFFPKDPWYCNYVQICAPNGRIYHFPAYQWMDGYETLALREATGKTTADDSLPVLLEHRKEEIRAKQDFYHWRVFLPGLPSYVHIPSYRPPVRRHRNPNRPEWNGYIPGFPILINFKATKFLNLNLRYSFLKTASFFVRLGPMALAFKVRGLLDCKHSWKRLKDIRKIFPGKKSVVSEYVAEHWAEDTFFGYQYLNGVNPGLIRRCTRIPDKFPVTDDMVAPFLGEGTCLQAELEKGNIYLADYRIMEGIPTVELSGRKQHHCAPLCLLHFGPEGKMMPIAIQLSQTPGPDCPIFLPSDSEWDWLLAKTWVRYAEFYSHEAIAHLLETHLIAEAFCLALLRNLPMCHPLYKLLIPHTRYTVQINSIGRAVLLNEGGLSAKGMSLGVEGFAGVMVRALSELTYDSLYLPNDFVERGVQDLPGYYYRDDSLAVWNALEKYVTEIITYYYPSDAAVEGDPELQSWVQEIFKECLLGRESSGFPRCLRTVPELIRYVTIVIYTCSAKHAAVNTGQMEFTAWMPNFPASMRNPPIQTKGLTTLETFMDTLPDVKTTCITLLVLWTLSREPDDRRPLGHFPDIHFVEEAPRRSIEAFRQRLNQISHDIRQRNKCLPIPYYYLDPVLIENSISI

SEQ ID NO: 29 - protein, 662 aa, Homo sapiens
MGLYRIRVSTGASLYAGSNNQVQLWLVGQHGEAALGKRLWPARGKETELKVEVPEYLGPLLFVKLRKRHLLKDDAWFCNWISVQGPGAGDEVRFPCYRWVEGNGVLSLPEGTGRTVGEDPQGLFQKHREEELEERRKLYRWGNWKDGLILNMAGAKLYDLPVDERFLEDKRVDFEVSLAKGLADLAIKDSLNVLTCWKDLDDFNRIFWCGQSKLAERVRDSWKEDALFGYQFLNGANPVVLRRSAHLPARLVFPPGMEELQAQLEKELEGGTLFEADFSLLDGIKANVILCSQQHLAAPLVMLKLQPDGKLLPMVIQLQLPRTGSPPPPLFLPTDPPMAWLLAKCWVRSSDFQLHELQSHLLRGHLMAEVIVVATMRCLPSIHPIFKLIIPHLRYTLEINVRARTGLVSDMGIFDQIMSTGGGGHVQLLKQAGAFLTYSSFCPPDDLADRGLLGVKSSFYAQDALRLWEIIYRYVEGIVSLHYKTDVAVKDDPELQTWCREITEIGLQGAQDRGFPVSLQARDQVCHFVTMCIFTCTGQHASVHLGQLDWYSWVPNAPCTMRLPPPTTKDATLETVMATLPNFHQASLQMSITWQLGRRQPVMVAVGQHEEEYFSGPEPKAVLKKFREELAALDKEIEIRNAKLDMPYEYLRPSVVENSVAI

SEQ ID NO: 30 - protein, 937 aa, Physcomitrella patens
MMLNRLETGSLASAFRGSREEFVVSRGRSPGRSQSIQVRASSGGDPAGWLQTASKQLGKLSSFGEKRKTATSTSTRGPSGDNVQYTGVATTMKKLKVLDLIDRVADIQDDTSEIVGGKRVTVQLVSKDVDPKTGESMKSSEVIFPNWAGLEGPAASLIDFVLEFTVPKSFGVPGAILVKNAHPNEFLLVSFELELHDKSKAHYVTNSWVYNTEKTGARIFFQNTAYLPDETPASLKALREQELINLRGDGTGERQIGDRIYDYAVYNDLGNIEQNEKFERPNLGGNDMYHFPRRMRTGRRNTTVEAKKFPGMVYETRKTKGDFYIPRDEAFERAKMSDFLADGFRSIGHSVSSKVTGFVTRKQEFDTVEEIKKLYAKKGEKVGGINNVLPDKEDIPEQEQYPLVFLQEVLKPDGKMEHPLLYPLPQLLQADDTSWRSNDEFAREFLAGLNPVMITRVKFPIRSSLDPAEFGDPTSAITKDHIEGSLEGLSVEEAVTSNRLFVVDYHDAFLPFVAKINAQQNSATYATRTLLFLSKDGILKLLAIELALPPKTVGEERITRVLTTRKDDQLWKVNWEWELAKAHVSNNDITAHQVFSHFSRCHAVTEAVIICSNRNLSKLHPLMQLLAPHFKSTLEINRQARATLIAAGGSIETHFTTRAYSLEMAAVNYKDTWTFESQALPTDLVARGMAVPDPDSPHGVRLVVEDYPYAADGLELWGALKAWHKEYVDIYYKDDAAVLQDSELMTWWTEMREKAHEDKKDSHGWPELNSKEALVDILTTVIWIPSCLHAAVNFGQYDFAGFMPHHPTLTRRLLPEHGNEKDKADFNKNPEKYYLTSISNIDSTTTAMSVYEVLSAHCPIEEYIGERRGNWTNNEKVLAAFKGFKESVNEADAVMRARNADPKLRNRGGPVKMPYQLLRPHSKPGVTSMGVPNSITI

SEQ ID NO: 31 - protein, 676 aa, Homo sapiens
MAEFRVRVSTGEAFGAGTWDKVSVSIVGTRGESPPLPLDNLGKEFTAGAEEDFQVTLPEDVGRVLLLRVHKAPPVLPLLGPLAPDAWFCRWFQLTPPRGGHLLFPCYQWLEGAGTLVLQEGTAKVSWADHHPVLQQQRQEELQARQEMYQWKAYNPGWPHCLDEKTVEDLELNIKYSTAKNANFYLQAGSAFAEMKIKGLLDRKGLWRSLNEMKRIFNFRRTPAAEHAFEHWQEDAFFASQFLNGLNPVLIRRCHYLPKNFPVTDAMVASVLGPGTSLQAELEKGSLFLVDHGILSGIQTNVINGKPQFSAAPMTLLYQSPGCGPLLPLAIQLSQTPGPNSPIFLPTDDKWDWLLAKTWVRNAEFSFHEALTHLLHSHLLPEVFTLATLRQLPHCHPLFKLLIPHTRYTLHINTLARELLIVPGQVVDRSTGIGIEGFSELIQRNMKQLNYSLLCLPEDIRTRGVEDIPGYYYRDDGMQIWGAVERFVSEIIGIYYPSDESVQDDRELQAWVREIFSKGFLNQESSGIPSSLETREALVQYVTMVIFTCSAKHAAVSAGQFDSCAWMPNLPPSMQLPPPTSKGLATCEGFIATLPPVNATCDVILALWLLSKEPGDQRPLGTYPDEHFTEEAPRRSIATFQSRLAQISRGIQERNQGLVLPYTYLDPPLIENSVSI

SEQ ID NO: 32 - protein, 685 aa, Pseudomonas aeruginosa
MKRRSVLLSGVALSGTALANDSIFFSPLKYLGAEQQRSIDASRSLLDNLIPPSLPQYDNLAGKLARRAVLTSKKLVYVWTENFGNVKGVPMARSVPLGELPNVDWLLKTAGVIVELIVNFVASLPASAAAQFERIATGLSGDLEAARQVHEALLEEAKNDPAAAGSLLLRFTELQTRVIAILTRVGLLVDDILKSASNLVTQRGQGDGLNRFRAVFGTLRLPEVADSFRDDEAFAYWRVAGPNPLLIRRVDALPANFPLGEEQFRRVMGADDSLLEAAASRRLYLLDYAELGKLAPSGAVDKLLTGTGFAYAPIALFALGKDRARLLPVAIQCGQDPATHPMFVRPAESESDLYWGWQMAKTVVQVAEENYHEMFVHLAQTHLVSEAFCLATQRTLAPSHPLHVLLAPHFEGTLFINEGAARILLPSAGFIDVMFAAPIQDTQATAGGNRLGFDFYRGMLPESLKARNVDDPLALPDYPYRDDGLLVWNAIRQWAADYVAVYYASDGDVTADVELAAWVGEVIGSGKVAGFRPITGRSQLVEVLTMVIFTASAQHAAVNFPQPSMMTYAPAICAMSAAPAPDSPSGKSEADWLKMMPPTLVALEKVNIYHLLGSVYHGRLGDYRQTGFPYAPVFSDRRVTASGGPLERFQARLKEVEATIRTRNQARRRPYEYLLPSRIPASTNI

SEQ ID NO: 33 - protein, 569 aa, Cyanothece sp. [sequence omitted]

SEQ ID NO: 34 - protein, 630 aa, Nostoc punctiforme
MTALSPDHSISSSSTHTLDIARQEYQYNYNHIPSIAMVDRLSITEEFTTNWYFLLAQQLRVLFINTLIVNRGNQDSKSIRDDVERFILEALLKGAVPARISILARILQIIPQLLLKEISKDFRELDDLFHSILKENGLAILRDALKRIITLLYEGQPTGHATSLKDYENLFPVISLPAIAKTYQEDEVFAYMRVAGYNPVTIKRVTTLSDRFPVTDEHYQAVMGTDDSLAAAGIEGRLYLADYKILDGAINGTFPHEQKYLYAPLALFALPKGSDPTRLLRPVAIQCGQTPGPDYPIVTPNSGKYAWLFAKTIVQIADANIHEAVTHLARTHLLVGVFAIATARQLPLTHPLRILLRPHFDSTLAINDAAQRILIAPGGGVDRLLSSSIDNSRVLAVLGLQSYSFNSTILPNQFQQRGVDDPNLLPIYPYRDDALLIWNAIHQWVWDYLNLYYTTDEDIQKDRALQAWAAEIPAYDGGRIPDFGEDGGIKTLNYLIDATTLIIFTASAQHAAVNFPQKDLMGYAAAIPLAGYLPASTLKREVTEQDYLNLLPPLDQAQRQYNLLSLLGSVYYNKLGEYEQGYFTDEKVKPLLQAFQSHLQQVENTIKQRNLHRPPYEYLLPSKIPQSINI

SEQ ID NO: 35 - protein, 936 aa, Hordeum vulgare
MLTATKPLVGGACAAPSSSARRRTFVVPEARRKPGNGRRTSVSKVGSTSTSTTTTTTTTLSADSNGAAVGTVTRPDVHVQDRTHATEMKATVTVHMSKAAGVRDFLYDLILKTWLHVDLVSSELDPQTGQEREPISGAVKHSGRVDDEWDMYEATFKVPASFGPIGAVQVTNYHHSEMLLGDIEVFPTGQEESAVTFHCKSWIDPSHCTPDKRVFFPAHSYLPSQTPKGVEGLRKRELEILRGTGCGERKEHDRIYDYDVYNDLGNPDDDNNPTTRPVLGGKEHPYPRRCRTGRPRSKKDPFSEERSHKEHIYVPRDEAFTERKMGAFDTKKFMSQLHALTTGLKTAKHKSQSFPSLSAIDQLYDDNFRNQPVQPEGGKLRFVIDLLETELLHLFKLEGAAFLEGIRRVFKFETPEIHDRDKFAWFRDEEFARQTIAGMNPMSIQLVTEFPIKSNLDEATYGPADSLITKEVVEEQIRRVMTADEAVQNKKLFMLDYHDLLLPYVHKVRKLDGTTLYGSRALFFLTADGTLRPIAIELTRPKSKKKPQWRQVFTPGCDGSVTGSWLWQLAKAHILAHDAGVHQLVSHWLRTHACTEPYIIAANRQLSQMHPVYRLLHPHFRFTMEINAQARAMLINAGGIIEGSFVPGEYSLELSSVAYDQQWRFDMEALPEDLIRRGMAVRNPNGELELAIEDYPYANDGLLVWDAIKQWALTYVQHYYPCAADIVDDEELQAWWTEVRTKGHADKQDEPWWPELDSHENLAQTLATIMWVTSGHHAAVNFGQYPMAGYIPNRPTMARRNMPTEIGGDDMRDFVEAPEKVLLDTFPSQYQSAIVLAILDLLSTHSSDEEYMGTHEEPAWTKDGVINQAFEEFKESTRKIVEQVDEWNNDPDRKNRHGAGMVPYVLLRPSDGDPTDGDPTDEKMVMEMGIPNSISI

SEQ ID NO: 36 - protein, 639 aa, Arabidopsis thaliana
MKVITSLISSILLKFIHKDFHEIYARMSLLDRFLLLIVHGVDKMVPWHKLPVFLGLTYLEVRRHLHQQYNLLNVGQTPTGIRFDPANYPYRTADGKFNDPFNEGVGSQNSFFGRNCPPVDQKSKLRRPDPMVVATKLLGRKKFIDTGKQFNMIAASWIQFMIHDWIDHLEDTHQIELVAPKEVASKCPLSSFRFLKTKEVPTGFFEIKTGSQNIRTPWWDSSVIYGSNSKTLDRVRTYKDGKLKISEETGLLLHDEDGLAISGDIRNSWAGVSALQALFIKEHNAVCDALKDEDDDLEDEDLYRYARLVTSAVVAKIHTIDWTVQLLKTDTLLAGMRANWYGLLGKKFKDSFGHAGSSILGGVVGMKKPQNHGVPYSLTEDFTSVYRMHSLLPDQLHILDIDDVPGTNKSLPLIQEISMRDLIGRKGEETMSHIGFTKLMVSMGHQASGALELMNYPMWLRDIVPHDPNGQARPDHVDLAALEIYRDRERSVPRYNEFRRSMFMIPITKWEDLTEDEEAIEVLDDVYDGDVEELDLLVGLMAEKKIKGFAISETAFYIFLIMATRRLEADRFFTSDFNETIYTKKGLEWVNTTESLKDVIDRHYPDMTDKWMNSESAFSVWDSPPLTKNPIPLYLRIPS

SEQ ID NO: 37 - protein, 631 aa, Arabidopsis thaliana
MGFSPSSSWFLHPQLHHVVSKMSYFDAFLFYIVHLVDKLGLWHRFPVLLGVAYLGLRRHLHQRYNLVHVGPINGQGYDTDEFCYRTADGKCNHPSDNTIGSQGSFIGRNMPPSTSQYGILDPHPSVVATKLLARKRFIDNGDQFNVIACSWIQFMIHDWVDHLEDTHQIELEAPEEVASGCPLKSFKFLRTKKVPTDDHHKSGAVNTRTPWWDGSVIYGNDETGMRRVRVFKDGKLKISGDGLLERDERGVPISGDIRNSWSGFSLLQALFVKEHNSVCDMLKERYPDFDDEKLYRTARLVTAAVIAKVHTIDWTIELLKTDTLTAGMRINWYGFFGKKVKDMVGARFGPLFSGLVGLKKPNDHGVPYSLTEEFVSVYRMHCLLPETLILRDMNSENVDKENPAIEREIPMTELIGKKAGEKASKLGFEQLLVSMGHQSCGALTLWNYPNWMRNLVAQDIDGEDRPHLIDMAALEIYRDRERGVPRYNEFRKNLLMSPISKWEELTDDEEAIKVLREVYEDDIEKLDLNVGLHAEKKIKGFAISETAFFIFLLVASRRLEADRFFTTNFNEKTYTKEGLEWVNTTETLKDVIDRHFPRLTDQWMRCSSAFSVWGSDPNPKNWVPLYLRSAP

SEQ ID NO: 38 - protein, 613 aa, Fusarium graminearum
MASVTSIIFVALVAGVLYAARMSLVPILKSLYIRLWKGVNHFIEWHKLPTWFAVFNLLALRYELREGNLHDTSPNAEFQGTDKCPMSDSKFVSSRDSDGLYNDLKQPKMGCAGMRFGRNVPRKYTKPPTEQELLTPNPRVISEKILARPEGQFKPAEIVNLLAAAWIQFQVHDWAQHFLVTNGDKDIDIPLHNKDKWTEQSMKIPRTKKADILSKQDAETPAYDNENTHWWDASQIYGSSEAETQALRAKCHKSKPGQLELHLSNPSWSSDHIFDTARLINCALMAKIHTVEWTPGILQHPALQIGMNANWWGLLGDKLWHAFGRVFDNKSEVISGIPGSGVDHDKAPYCLTEEFVSVYRLHSLIPDNVAFFNIKDGQHEGTLPIVDVSFESARKPFDEGKSGLGLSFADVFYSFGVNYPGAIRAHNMPNFLRDLKIPADKDFPEGRHLDLGTIDILRDRERGVPRYNAFRRLFHMPAAKSFIDLTGGDDKLASELEEVYEGDLEAVDLLVGTLCEPLPKGFGFSDTAFRVFILMATRRIKSDRFIAGDGWCPEVYTREGMDWVQKNTMKDVLCRHFPELAAPLHNVKNAFAPWTKLGQTAAYAGPETNKAKS

SEQ ID NO: 39 - protein, 653 aa, Fusarium verticillioides
MASVLSKESLAIILSVVTLLIGLSHFNMISLKSIFKSVYIRLWKLVNVFVHWHKLPTWLGVFNLLALRYELREKNLHDTYPNAEFQGTAADCPMKNSKFIATRNSDGDFNDLAQPKMGCAGMRFGRNVPRNHTTPPTQQELLTPNPRLISEKILARPEGQFKPAEIVNLLAAAWIQFQVHDWAQHSLVTNGDKDVEILLDKADRWSERIMKIPRTKKDDPLSQQDIETPAYTNECTHWWDASQIYGSTEAETKALRAQCDKSYPGQLHVTREDGVQFLPRSDDGIPKTGFRQNWWLGLELLHTLFALEHNAIATQLHLSNPSWSSDQIFDTARLINCALMAKIHTVEWTPGILQHPALQIGMNANWWGLLGDKLWHVFGRVFDNKSEVISGIPGSGVDHDNVPYCLTEEFVSVYRLHPLIPDNVAFFSIKDGQHKGTLPIKEVAFKSARKPFDEDKSGLGLSFADVFYSFGVNYPGAIRAHNMPNFLRDLNIPGDKDFPHGRHLDLGTIDILRDRERGVPRYNAFRRLFHMAPAKTFIDLTGGDSKLAAELEEVYDGDLEAVDLLVGTLSEPLPKGFGFSDTAFRVFILMATRRIKSDRFLAGDGWCPEVYTREGINWVQNNTMKDVLCRHFPELAATLHNVKNLSVSFILSL

SEQ ID NO: 40 - protein, 668 aa, Fusarium oxysporum
MASVLSKESLAISLSIVTLLIGLSHFNMISLKPIFKSVYIRLWKFVNIFVHWHKLPTWLGVFNLLALRYELREKNLHDTYPNAEFQGTTADCPMKNSKFIANRNSDGDFNDLAQPKMGCAGMRFGRNVPRKYTTPPTQQELLTPNPRIISEKILARPEGQFKPAEIVNLLAAAWIQFQVHDWAQHFLVTNGDKDVEIPLDKADRWSERIMKIPRTKKDDALSQQDIETPAYTNECTHWWDASQIYGSTEAETKALRAQCDKSYPGQLHVTREDGVQFLPRSDDGIPKTGFRQNWWLGLELLHTLFALEHNAIATQLHLSNPSWSSDQIFDTARLINCALMAKIHTVEWTPGILQHPALQIGMNANWWGLLGDKLWHVFGRVFDNKSEVISGIPGSGVDHDNVPYCLTEEFVSVYRLHPLIPDNVAFFSIKDGQHKGTLPIKDVAFESARKPFDEDKSGLGLSFADVFYSFGVNYPGAIRAHNMPNFLRDLNIPGDKDFPQGRHLDLGTIDILRDRERGVPRYNAFRRLFHMAPAKSFLDLTGGDAKLAAELEDVYDGDLEAVDLLVGTLSEPLPKGFGFSDTAFRVFILMATRRIKSDRFLAGDGWCPEVYTREGINWVQNNTMKDVLCRHFPELAATLHNVKNAFAPWTKIGQTEAYAGPETNKAKN

SEQ ID NO: 41 - protein, 618 aa, Oryza sative
MGSGLFKPRVHPDLRDVFSKMSFFDKIGFLFIHAFDKRNLWHKVPVPIGLLYLNTRRTLLEKYNLLAVGRSSHGALFDPKEFLYRTEDGKYNDPHNAEAGSQNTFFGRNMEPVDQQDELMSPDPFVVATKLLARREYKDTGKQFNILAAAWIQFMVHDWMDHMEDTGQIGITAPKEVANECPLKSFKFHPTKELPTNSDGIKIGHYNIRTAWWDGSAVYGNNEERAEKLRTYVDGKLVIGDDGLLLHKENGVALSGDIRNSWAGVSILQALFVKEHNAVCDAIKEEHPNLSDEELYRYAKLVTSAVIAKVHTIDWTVELLKTKTMRAAMRANWYGLLGKKIKDTFGHIGGPILGGLVGLKKPNNHGVPYSLTEEFTSVYRMHSLIPSTLKLRDPTGQPDANNSPPCLEDIDIGEMIGLKGEEQLSKIGFEKQALSMGYQACGALELWNYPSFFRNLIPQNLDGTNRSDRIDLAALEVYRDRERSVPRYNEFRRRLFLIPIKSWEDLTSDKDAIETIRAIYGDDVEKLDLLVGLMAEKKIKGFAISETAFNIFILMASRRLEADRFFTSNFNEETYTKKGMQWVKTTEGLRDVINRHYPEITAKWMKSSSAFSVWDADY

SEQ ID NO: 42 - protein, 599 aa, Homo sapiens
MSRSLLLWFLLFLLLLPPLPVLLADPGAPTPVNPCCYYPCQHQGICVRFGLDRYQCDCTRTGYSGPNCTIPGLWTWLRNSLRPSPSFTHFLLTHGRWFWEFVNATFIREMLMRLVLTVRSNLIPSPPTYNSAHDYISWESFSNVSYYTRILPSVPKDCPTPMGTKGKKQLPDAQLLARRFLLRRKFIPDPQGTNLMFAFFAQHFTHQFFKTSGKMGPGFTKALGHGVDLGHIYGDNLERQYQLRLFKDGKLKYQVLDGEMYPPSVEEAPVLMHYPRGIPPQSQMAVGQEVFGLLPGLMLYATLWLREHNRVCDLLKAEHPTWGDEQLFQTTRLILIGETIKIVIEEYVQQLSGYFLQLKFDPELLFGVQFQYRNRIAMEFNHLYHWHPLMPDSFKVGSQEYSYEQFLFNTSMLVDYGVEALVDAFSRQIAGRIGGGRNMDHHILHVAVDVIRESREMRLQPFNEYRKRFGMKPYTSFQELVGEKEMAAELEELYGDIDALEFYPGLLLEKCHPNSIFGESMIEIGAPFSLKGLLGNPICSPEYWKPSTFGGEVGFNIVKTATLKKLVCLNTKTCPYVSFRVPDASQDDGPAVERPSTEL

SEQ ID NO: 43 - protein, 624 aa, Pseudomonas aeruginosa
MHPTFSRVLLAAALAAAGSPAVATEIQLEQGWNAEQRASWYDASLGSRLLPLAWAQALERPDSEERLFSEDNARRLGFPLRNWQGGELRLPRGFALDQQDDSQFSDTRLRWKARQSSSEPWVGLNCAGCHSTDISYRGSELTVDAGATLANVQAIFDEVLAALRRTSDDGDKFARFAGNVLGSEDSPANRELLKAALVKRAALIDTLLSMSATDLQPGPGRLDATGQSLNRAAINSGARHLQANPTDAPTSFPALWHTLQMDKLQSSGFVPNVKVLDLNGQVFDLGYLAGDIGVVQGDYGDVVSHPLSGLEGYISSIRVDNLTRVEGLIHKLKAPAWPSQLFGAPDSARLAQGKRLYEENCAACHASIGRDDLQTPIKVRQVRLKAHGDDAPIGTDPWMACNTFTFSSPSGNYFGLFRPSLGTPSGVGIVGRTSKIADMQVPEVFQIMLGKKGQLADGIAEIIHAIVTGQQTLPGSDSLQAVPAGQLLLAGAAPADSQAQSLAAGEVPTDKSARKDYCLNTEHPFLGYIARPLNGIWATAPYLHNGSVPSLYDLLLPQEQRPATFYTGSHEFDPSRVGYLTAPGPDNAFLFDTHLEGNSNAGHDFAREYDESQRLALLEYLKTL

SEQ ID NO: 44 - protein, 624 aa, Pseudomonas aeruginosa
MHPTFSRILLAAALASAGSPAVATEIQLEQGWNAEQRASWYDASLGSRLLPLAWAQALERPDSEERLFSEDNARRLGFPLRNWQGGELRLPRGFALDQQDDSQFSDTRLRWKARQSSSEPWVGLNCAGCHSTDISYRGSELTVDAGATLANVQAIFDEVLAALRRTSDDGDKFARFAGNVLGSEDSPANRDLLKAALAKCAALIDTLLSMSATDLQPGPGRLDATGQSLNRAAINSGARHLQANPTDAPTSFPALWHTLQMDKLQSSGFVPNVKVLDLNGQVFDLGYLAGDIGVVQGDYGDVVSHPLSGLEGYISSIRVDNLTRVEGLIHKLKAPAWPSQLFGAPDSARLAQGKRLYEENCAACHASIGRDDLQTPIKVRQVRLKAHGDDAPIGTDPWMACNTFTFSSPSGNYFGLFRPSLGTPSGVGIVGRTSKIADMQVPEVFQIMLGKKGQLADGIAEIIHAIVTGQQTLPGSDSLQALPTGQLLLAGGDPAGSQAPSLAAGEVPADKSARKDYCLNTEHPFLGYIARPLNGIWATAPYLHNGSVPSLYDLLLPQEQRPTTFYTGSHEFDPSRVGYLTGPGPDNAFLFDTHLEGNSNAGHDFAREYDESQRLALLEYLKTL

SEQ ID NO: 45 - protein, 711 aa, Homo sapiens
MAVYRLCVTTGPYLRAGTLDNISVTLVGTCGESPKQRLDRMGRDFAPGSVQKYKVRCTAELGELLLLRVHKERYAFFRKDSWYCSRICVTEPDGSVSHFPCYQWIEGYCTVELRPGTARTICQDSLPLLLDHRTRELRARQECYRWKIYAPGFPCMVDVNSFQEMESDKKFALTKTTTCVDQGDSSGNRYLPGFPMKIDIPSLMYMEPNVRYSATKTISLLFNAIPASLGMKLRGLLDRKGSWKKLDDMQNIFWCHKTFTTKYVTEHWCEDHFFGYQYLNGVNPVMLHCISSLPSKLPVTNDMVAPLLGQDTCLQTELERGNIFLADYWILAEAPTHCLNGRQQYVAAPLCLLWLSPQGALVPLAIQLSQTPGPDSPIFLPTDSEWDWLLAKTWVRNSEFLVHENNTHFLCTHLLCEAFAMATLRQLPLCHPIYKLLLPHTRYTLQVNTIARATLLNPEGLVDQVTSIGRQGLIYLMSTGLAHFTYTNFCLPDSLRARGVLAIPNYHYRDDGLKIWAAIESFVSEIVGYYYPSDASVQQDSELQAWTGEIFAQAFLGRESSGFPSRLCTPGEMVKFLTAIIFNCSAQHAAVNSGQHDFGAWMPNAPSSMRQPPPQTKGTTTLKTYLDTLPEVNISCNNLLLFWLVSQEPKDQRPLGTYPDEHFTEEAPRRSIAAFQSRLAQISRDIQERNQGLALPYTYLDPPLIENSVSI

SEQ ID NO: 46 - protein, 393 aa, Nostoc punctiforme
MKLFTEYPEKDELKYCDLMSELVKKNMENLYGGKKKKTAKRDTHSKTHAAVQGTLEIFDFDEAAIKQELSKRTSLSEAELSAISLKQGLFATPKQYPVWLRFANGAFSVKNDYEGDTRSMAVKAIGVEGERLSQSHELKTQDIITHNTEFFFVRTIKDFHSFFLTVYRAGLFPLFKLLVLFWLKLHPYESTLLQTSFKRFPKSLLKERYWSASAFSVGLKSGFDPSQPGRVPVEYPAVIKYGFTPVSSQPPHQQFPLESRSESELKLAKASGSEDNYYREDIIQALAKPDAEYYWDFQIQFQTSPEMSIDDTTIVWNEEESPFFTVGRLTIKHQKVNYPQANDFGENLSFSPGNGLAVHRPVGAINRLRSIVYPIVANDRHQKRGVKYQEPTV

SEQ ID NO: 47 - protein, 1143 aa, Aspergillus terreus
MSSVIVALAVLVLSLLYLTLFRNDLTHLIIEKLQSFRTGSGWELSPRSRLLPRATKAALSSITGTGVGIWSRLYARIFHSDELAEEEDDEKYQAGEAYGDPKVLATSLIKDLRALGVKGRRSDLRTLIEMVKNKGKPMDDRQMHMEKIIAIVAMLPRTSKARQRLTGVLIDQLWRSLQHPPLSYFGNKYQYRTPDGSYNNPLEPNLGKAGSPYARSIPRIKTMHGVRPDPGLLFDLLMARDDSTFKENPAGISSMLFYHASIIIHDIFRTNRRDPNISDTSSYLDLAPLYGSSLEDQLKVRTMEKGMLKPDTFHEKRLLGQPAGVNVILVMYSRFHNYVADMLLKINENGRFTLPPTSSEEARKKALAKQDEDLFQVARLVVNGLYVNISLHDYLRGLTNTHHSASDWTLDPRIAVGRTFDPDGVPRGIGNQISAEFNLLYRFHSVISRRDEKWTNEFLKSLFPDLNKPLDQLTPQEFMMGLMRYEQSIDKDPSKREFGGLKRSPDGKFNDADLVQILKDSMEDPAGLFGPRNVPKALRMIEIAGIMSARKWDLGSLNEMRDFFKLKRHATFEDINPDPEIADLLRKLYDHPDMVEMYPGMFLEDAKPRLDPGCGGCPPYTVGRAVFSDAVTLVRSDRFLTLDYTASNLTNWGFREVQQDYDILGGSMFHKLIQRALPGWFPYNSLHATQPMFTRKMNEQIAREIGTIDHYSLADPAPPPRKIVLTDYATNIKVLKDQASFRVPWARYLNDMFPGKTYNDYMLGGDDPANAAQKKLVHSILFSPDQFLDLLSETTTKLGSELLKANTLWLTKDLHQVDIIRDVAIPLNARIMADLFCLDMKTPENPTGSMNAATVYRHLMNVRIWGFNNNDPALMLQRRKWAIESAEALIETTRKLVNEQAQPAQSGVLKNLMTRRQATGTLRWYGNNVAKEMMEMGMSAEEVADICWLTAIGGVGTPSGVVANVLQYYFRYENIGHWEEIQKLVTQPDTPAADRTLRQYVLEANRLTSMECTVRVCARPVTVDGHDFKPGEVIVNHLGLACRDPHNIPDADKFRLDRPASAYIQWGYGAHECLGKEIAITFAVSMIRILAGLKYLRPAPGEMGVLKSVMADGRQAFLNDSWSWLTQDPTSKSNMHGKASAVD

SEQ ID NO: 48 - protein, 518 aa, Arabidopsis thaliana
MASISTPFPISLHPKTVRSKPLKFRVLTRPIKASGSETPDLTVATRTGSKDLPIRNIPGNYGLPIVGPIKDRWDYFYDQGAEEFFKSRIRKYNSTVYRVNMPPGAFIAENPQVVALLDGKSFPVLFDVDKVEKKDLFTGTYMPSTELTGGYRILSYLDPSEPKHEKLKNLLFFLLKSSRNRIFPEFQATYSELFDSLEKELSLKGKADFGGSSDGTAFNFLARAFYGTNPADTKLKADAPGLITKWVLFNLHPLLSIGLPRVIEEPLIHTFSLPPALVKSDYQRLYEFFLESAGEILVEADKLGISREEATHNLLFATCFNTWGGMKILFPNMVKRIGRAGHQVHNRLAEEIRSVIKSNGGELTMGAIEKMELTKSVVYECLRFEPPVTAQYGRAKKDLVIESHDAAFKVKAGEMLYGYQPLATRDPKIFDRADEFVPERFVGEEGEKLLRHVLWSNGPETETPTVGNKQCAGKDFVVLVARLFVIEIFRRYDSFDIEVGTSPLGSSVNFSSLRKASF

SEQ ID NO: 49 - protein, 1066 aa, Plexaura homomalla; identical to SEQ ID NO: 26

SEQ ID NO: 50 - protein, 1151 aa, Fusarium oxysporum
MSFNEKFQAGESYGDSKEDPSSLLNNPEKLVADLMKDFAGVRSQASPAQLLGLVKELLQKGQPLDDKKGTTELLIGILTALPATSKARTALTNKLIDTLWGNLQHPPLSYMGGDVKYDVVNSDKPAHKHNCELYDTIEFKVPGTDVLLREQVPQAPDGLHQYRMPDGSFNNILEPNLGRAGTPYAKSVKSEKRLHGVKPDPGLLFDLLMARDETTFQENPAGISSMLFYHAAIIIHDIFRTNRTDMNKSDTSSYLDLAPLYGSSLKDQHEIRTMKEGKLKPDTFHEKRLLGQPAGVNVMLVLYSRFHNYVADILLKINENGRFSLSVPPNASEEDKAKAIAKQDHDLFNVARLITGGLYINICLHDYLRAITNTHHSASDWTLDPRVAIDKQFDGDGVPRGVGNQVSVEFNLLYRFHSCISKRDEKWINNFFLKLFPGRKAEDLQDVSWTELGQALLIFEQNTPKDPSVRTFDGLERQADGTFKDEDLVRILKDAMEDPAGTFGARMVPKALKVVEVLGIIQGRKWQCASLNEFREFFGLKRYDSFSEINSNPDIANILEKLYTDPDMVELYPGLMIEDIKPQRNPGSGIMPTYSVGRAVLSDAVTLVRSDRFNTIDYTVSNLTAWGYNEVQQDYKTLGGSMLYKLIQRGVPNWFPFNSIAVMQPMYTKKANEQIAKEIGTFDQYTLDDPKAPPKVAVLTSGPAIKQILSNTKQYVVPWLKPLNTLFPGKKDFGWFMLAGDQPQNYTHRANFSKAMSKIPNMHNAVHAFIEREGTKLINKETFTLKKGLDQIDIIRDVAIPLNTQLLADLFYFDLRTEENPDGKLGVAELYRSLLDIRIWGVNNNDPAQAWNRRRRAQEGAKRMIETTKTIVAEADAGRPRGIGLVSAVANRIGARSYLKKDSLRSCGLKLVEELLAQGNNVDQVTDNLWLTAFGGIGVPVTAFYEVLSFFLRPENEAIWAEVQAIAQKGDDATLHAYVAEAQRMTSSQRNVRVATAPGEVQGQAIQPGTAVVLMLGEAGRNPKEVPDAGKFNPQRKKEDVSAFSYGQHECIAKDVALAFVTGLIKLVADLKELRPAPGQMGTVKTIQVGTEKAYLNDSWSYLGFDASTWKVHFNGHGKGKFEGERVPTKSTPIQEYYYLLQKRKDEILGN

SEQ ID NO: 51 - protein, 1162 aa, Colletotrichum graminicola
MSFDQKFMAGETYGDERKSSANFFSDPTKVATDLLKDYAGLRSQTSPAELAGLIKELLQKGQPLDDKKGTTEILIGILTSLPSTSSTRVQLTNKLIDTLWGTLQHPPLSYVGGDVKYEVVNPNETASKDKQQTEDSIEFKAPDSDVILREQVPRPPDGLHHYRMPDGSYNNILEPNLGKAGTPYAKTVRTSKRLHGVKPDPGLLFDLLMARDDSTFKENPAGISSMLFYHASIIIHDIFRTNRTDMNKSDTSSYLDLAPLYGSSLKDQLEIRTMKEGMLKPDTFHERRLLGQPAGVNAMLVLYNRFHNYVCDILLKINENGRFTLQCPADASPEDRAKAVAKQDHDLFNTARLIVGGLYINISLHDYLRAITNTHHSKSDWTLDPRVEIGKQFDGEGVPRGVGNQVSVEFNLLYRFHSCISKKDERWIDNFFAKLFPDRKPEDLQNVGMAELGQALMTFEQSIPKDPSARTFDNLERQADGKFKDEDLVRVLKEAMDDPAGCFGARMVPKALKIVEILGINQARKWQVASLNEFREFFGLKKYDKFAEINSNPEIATLLEKLYTDPDMVELYPGLMIEDIKPARNTGSGICPTYSVGRAVLSDAVTLVRSDRFNTLDYTVSNLTAWGYNEVQQDYKTLGGSMLYKLIQRGLPNWFPYNSVAVMQPMYTKKANESIAKELGTLHLYTSNDPKPPPKIVVVATSVAIKQVLGNSKQFVVPWLQPLNDLFTGTKKDISWFMLAGDEPKNYQHRVNLLKAMGKIPNLHNAVHEFVDRVGAKLIEKETFKLKEGLCQMDIIRDVAIPLNAQLLADLFYFDMRTDENPNGTLSAADLYRHLLNIRVWGVNNNDPAQAWNRRRRATESVNAIIDSTRGLVNEVVVGRGLGFGIASTISGVVGRKSNFKKDSLRSCGHKLVEELLAQGNSAEQVVDNMWLTAFGGIGAPVTAFYEVLEYFLRRENASIWAEVQTLAQKNDDAGLHAYVKEAQRLTSSQRNVRVATVAAEVDGKQVQPGNVVVMLLGDAGRNPKEVANPDKFDAKRKTDPVSAFSYGQHECLAKDIATTFIVGLVKLVADLKQLRPAPGQMGLVKTIRVGSEKAYLNDSWSYLGFDASTWKVHFDGHGKGNFEGDVQPNKPIDLGQYYYLLQKRKEKLLNGNSSNGTNGSS

SEQ ID NO: 52 - protein, 1161 aa, Glomerella cingulate
MAFNTKFQAGESYGDERKGSNNFFADPKKVAMDIIKDLGGAHGQLNLLEVTALVQQLLQKGEPLDDKKGTTEALIGILTSLPSGSNTRVQLTNKLIDTLWGNLQHPPLSYVGGDVKYEVVKTKEQLAKEQADLAAQGKAPQSPEESHITFKAPDFPDITLREHLPTPPDNYKMPDGSYNNILEPNLGAAGTPYAKTVKTEKRLAGVKPDPGLLFDLLLARDDKKFTENPAGISSMLFYHASIIIHDIFRTNRHDLNKSDTSSYLDLAPLYGSSFKDQLEIRTMKEGKLKPDTFHEKRLLGQPAGVNVMLVLSSRFHNYVADILLKINENGRFTLQTAKDAAPEDQAKAVAKQDHDLFNVARLVTGGLYINICLHDYLRAITNTHHSKSDWTLDPRVEIGKQFDGEGVPRGVGNQVSVEFNLLYRFHSCISKKDERWIDGFFAKLFPGRKPEDLQNVGMEELGAALMKFEMGIDKDPSKRTFDDLQRGEDGKFRDEDLVRVLKEAMEDPAGTFGARMVPKALKIVEIMGIKQARAWQVASLNEFRDFFGLKRHDTFKDINSNEEIATLLEKLYTDPDMVELYPGLMIEDIKPVRNTGSGICPTYSVGRAVLSDAVTLVRSDRFNTIDYTVSNLTAWGYNEVQQDYKTLGGSMLYKLIQRGLPGWFPFNSIAVMQPMYTKKANERIAREIGTFNQFTLDDPKAPPKPVVVASSEGIKRVLGSPDKFVVPWLTPLNALYTDTKKDISWFMLAGDGSTNKQEKVNFVNAMKKVPNLHNAVHQFIERVGRQLIEKETFKLKEGLCQMDIIRDVAIPLNAQLLADLFYFDLRHEENPGGTLSATDLYRHLLNIRIWGVNNNDPGQAWNRRRRAAESAKVITDSTRKLVDEVSRGRGLNLGFISAINEVASRKTHIKKDSLRSCGYKLVEELLNQGGSPEKVTDNVWLTAFGGIGVPVTTFYEVMEYFLRPENKSIWGEVQALAQKNDEAGLHAYVNEAMRLTSGQRNVRIATVKDEIDGQKVEPGNAVVMLLGAAGRNPKEVPNADKFDAKRSTDHIKPFSYGQHECVGQDVARAFVTGLVKLVADLRQLRPAPGEMGKVKTIQVGTERAYLNDSWSYLGFDASTWKVHFDGHGQGTYEGDPEPNKPIDMGRYYYILQKRKESLLKG

SEQ ID NO: 53 - protein, 1251 aa, Aspergillus niger
MGSIFIALLLCLLSYLYLRVFADDLTRPLQILAKFFSSHQHPTWKLRPRFLPKATRAALSSIAGTGEGLWQRLYARTFHAQELAEVEDDLKYQAGEPYGDPDVLATGLVKDLSALGLKGKRSDLRTLIQLVKAKGKPIDDRQMLMEKVIAIVSMLPRTSKSRQRLTGILVDQLWQSLEHPPLSYFGNKYQYRTPDGSYNNPLEPDLGKAGSPYARSVPRLKALHGVQPDPGLLFDLLMARDDTTFRENPAGISSVLFYHASIIIHDVFCTNRRDPNISDTSSYLDLAPLYGSSYEDQLRVRTMQRGMLKPDTFHEKRLLGQPPGVNVILVMYNRFHNYVADVLLKINENGRFTLPPTTSEDAKRKALAKQDEDLFQVTRLIVNGLYVNISLHDYLRGLTNTHHSASDWTLDPRVAVSRAFDADGVPRGVGNQVSAEFNLLYRFHSVISRRDEQWTNEFLKSLFPDLKKPLEQLTPQEFMQGLINYERSIDKDPSKREFGGLKRNQDGRFNDAELVQILKDSMEDPAGLFGARMVPKALRMVEIAGILTARKWNLASLNEMRDFFKLKRHSSFEDINPDPKIADLLRKLYDHPDMVEMYPGIFLEDAKPAMDPGCGGCPPYTVGRAVFSDAVTLVRSDRFLTLDYTASNLTNWGIREVQQDYDILGGSMFHKLIQRALPGWFPYNSLHATQPMFTRKMNEQIAKEIGTIDRYSQEDPKPPPRTVMLANHATIIEVLKDQDTFRVPWARYLNDMIPGKRFNDYMLGGDGPVNAAQKKLVKSILFSPDQFNQLLSQTTVRLGKELLELNTLQLSKDLNQVDIIRDVAIPLNARIMADLFCLDMKTPENESGSMNAATVYKHLMNVRTWGFNNTDPGLMLQRRKWASESAEALVKTTLKVVNEQAQPQKTHMLKKLTGYQRSEVSTLRWYGNNVVKQMMEMDMTAAETAEVCWLTAVGGVGAPVGLVADVLQYYLRPENIDHWKRIQNLVSQPDNSGSIDKLLRQYVLEAQRLTSMECTVRVCRAHRTINDQEFKPGDVVITLLGPACRDPTSIPDAETFKLDRPSNAYIHFGYGAHECLGKEIGLTFAVSMLRVLAGLKYLRPAPGDMGMLKSIIVDGRRVYLNDSWSWMIQDPTTWKLHFAGYGQGAYEAPAPPPPAPTFPVIDQSPDTSDEDGVDDTIYSTVPTKHHHHGDPEYTRQESYTMTDGGIGMSTQYSFGQHHHHQYHEITRTSSSSLPSMLGDDESYGRFSGTLN

SEQ ID NO: 54 - protein, 478 aa, Solanum tuberosum
MSSYSELSNLPIREIPGDYGFPIISAIKDRYDYFYNQGEDAWFHNKAEKYKSTVVKINMAPGPFTSNDYKLVAFLDANSFVCMFDNSLIDKTDTLGGTFKPGKEYYSGYRPVAFIDTKDPNHAALKGYILSAFAKRHNLFIPLFRNSLSDHLFNNLEKQVTEQGKSDFNALLPTMTFNFIFRLLCDQTNPSDTVLGAQGPEHLRKWLFPQLIPSLSAKKLPNIIEDTLFHNFLIPFGFIKSDYNKLVDAFSKSAVSILDEAEKLGIKREEAVQNILFLVGINMFAGLNAFSPHLFRFVGEAGASLHTQLAKEIRTVIKEEGGAITLSAINKMSLVKSVVYETLRLRPPVPLQYGKAKKDFMVQSHDASYKINKGQFVVGYQPMASRDPKIFANPDEFVPDRFMNDGEKMLKHVLWSNGRETENPAPDNKQCPGKDLVHLLGRLILVEFFMRYDTFTVEITPLFRAPNVAFKTLTKASK

SEQ ID NO: 55 - protein, 472 aa, Allium sativum
MSTSNGSTENIQKPLRKIPDITGTPILTAIKDRLDFFYNQGQYEYFQSRVKKNNSTILRMNMIPGPFASNPKIVALCDAASFPTLFDPSKVSKVNSLTGNYMPALSFTGGYRVCAYLDPSEPTHTKIKQVFFNAQAAKKDTFIPTFVSTFNSMFDKMDAEVESKKKAEFTKFNEAAVFEFVGLALVGPKPAREVFDSAKKSVFFQFHPFITAGLPALVEELAFHMFPFPSFVAKSSYKILYEYFSTGGSWILDNAEEIGLSREEAIHHLIFTWAINAYLGIRTCLMRLFKWIVASGPDLQEKLAREVRSVVRSEEGKITFAGIEKMELVKSVAYESFRFDPPVQVQYGTAKSDLIIESHDGKYQVKKGEMLCGFQPMATRDPKVFDRADEFVPDRFMGDGKKLVKHVLWANGYGTDAPKADDKICAGKDLGVLVGRLLIAVMFLRYDKIGGVVGKTMEEVDVIVNELTKVAV

SEQ ID NO: 56 - protein, 1081 aa, Asperigullus nidalus
MGEDKETNILAGLGNTISQVENVVAASLRPLPTATGDGTYVAESTQTGLAKDLSHVDLKDVRTLAEVVKSAATGEPVDDKQYIMERVIQLAAGLPSTSRNAAELTKSFLNMLWNDLEHPPVSYLGADSMHRKADGSGNNRFWPQLGAAGSAYARSVRPKTMQSPSLPDPETIFDCLLRRKEYREHPNKISSVLFYLASIIIHDLFQTDPKDNSVSKTSSYLDLSPLYGNNQDEQNLVRTFKDGKLKPDCFATKRVLGFPPGVGVLLIMFNRFHNYVVDQLAAINECGRFTKPDESNVDEYAKYDNNLFQTGRLVTCGLYANIILKDYVRTILNINRTDSTWSLDPRMEMKDGLLGEAAAMATGNQVSAEFNVVYRWHACISKRDEKWTEDFHREIMPGVDPSTLSMQDFVAGLGRWQAGLPQEPLERPFSGLQRKPDGAFNDDDLVNLFEKSVEDCAGAFGASHVPAIFKSVEALGIMQARRWNLGTLNEFRQYFNLAPHKTFEDINSDPYIADQLKRLYDHPDLVEIYPGVVVEEAKDSMVPGSGLCTNFTISRAILSDAVALVRGDRFYTVDYTPKHLTNWAYNEIQPNNAVDQGQVFYKLVLRAFPNHFDGNSIYAHFPLVVPSENEKILKSLGVAEKYSWEKPSRISHPIFISSHAACMSILENQETFKVTWGRKIEFLMQRDKHQYGKDFMLSGDRPPNAASRKMMGSALYRDEWEAEVKNFYEQTTLKLLHKNSYKLAGVNQVDIVRDVANLAQVHFCSSVFSLPLKTDSNPRGIFAESELYKIMAAVFTAIFYDADIGKSFELNQAARTVTQQLGQLTMANVEIIAKTGLIANLVNRLHRRDVLSEYGIHMIQRLLDSGLPATEIVWTHILPTAGGMVANQAQLFSQCLDYYLSEEGSGHLPEINRLAKENTPEADELLTRYFMEGARLRSSVALPRVAAQPTVVEDNGEKLTIKAGQVVMCNLVSACMDPTAFPDPEKVKLDRDMNLYAHFGFGPHKCLGLDLCKTGLSTMLKVLGRLDNLRRAPGAQGQLKKLSGPGGIAKYMNEDQSGFTPFPSTMKIQWDGELPQLKEDF

SEQ ID NO: 57 - protein, 1079 aa, Aspergillus fumigatus
MSEKQTGSANGGLGKTLAQLEQVVSASLRPLPCQTGDGTYVTEQVKTGILKDLSHVDLGDLKTLVDVSKSALTGEALDDRKYIMERVIQLSAGLPSTSQIGKELTNTFLTTLWNDLEHPPISYLGRDAMYRRADGSGNNVLWPHIGAAGTPYARSVQPKTVQSPNLPDPETLFDCLLARKEYKEHPNKISSVLFYIASIIIHDLFETDRKDPAISLTSSYLDLSPLYGNNQQEQDLIRTFKDGKLKPDCFSTKRVLGFPPGVGVVLIMFNRFHNYVVEKLAMINEGGRFTKPQESDTAAYAKYDNDLFQTGRLVTCGLYVNIILKDYVRTILNINRTDSIWSLDPRSEMKDGLLGRAAAQATGNQVAAEFNLVYRWHSCISQRDQKWTEDMYQELFPGQDPSKISLQDFLRGLGRWEAKLPGEPRERPFAGLQRKADGSYDDNDLVKIFEESVEDCAGAFGALHVPTVFRSIEALGIQQARSWNLATLNEFRKYFNLAPYKTFEEINSDPYVADQLKRLYDHPDRVEIYPGIIVEDAKESMAPGSGLCTNFTISRAILSDAVALVRGDRFHTVDFTPKHLTNWAYNEIQPQDSVDQTHVFYKLVLRAFPNHFRGDSIYAHFPLVVPSENKKILTKLGTADKYSWDRPNYTPPPQFINSHSACMSILSDQETFKVTWGSKIEFLMRHNNQPYGRDFMLSGDRTPNAMSRQMMGKALYRDKWETEVKRFYENITLKLLHRYSYKLAGVNQVDVVRDIANLAQVHFCASVFSLPLKTESNPRGIFTESELYQIMAVVFTSIFYDADIGKSFELNQAARAVTQQLGQLTLANVELIAKTGFIANLVNSLHRHDVLSEYGVHMIQRLLDSGMPAPEIVWTHVLPTAGGMVANQAQLFSQSLDYYLSEEGSVHLPEINRLAKEDTTEADDLLLRYFMEGARIRSSVALPRVVAQPTVVEDNGQKITLKQGQHIICNLVSASMDPVTFPEPDKVKLDRDMNLYAHFGFGPHQCLGLGLCKTALTTMLKVIGRLDNLRRAPGGQGKLKKLSGPGGIAMYMTPDQTAFFPFPTTMKIQWDGDLPEVKE

SEQ ID NO: 58 - protein, 1153 aa, Magnaporthe oryzae
MDGAVRLDWTGLDLTGHEIHDGVPIASRVQVMVSFPLFKDQHIIMSSKESPSRKSSTIGQSTRNGSCQADTQKGQLPPVGEKPKPVKENPMKKLKEMSQRPLPTQHGDGTYPTEKKLTGIGEDLKHIRGYDVKTLLAMVKSKLKGEKLKDDKTMLMERVMQLVARLPTESKKRAELTDSLINELWESLDHPPLNYLGPEHSYRTPDGSYNHPFNPQLGAAGSRYARSVIPTVTPPGALPDPGLIFDSIMGRTPNSYRKHPNNVSSILWYWATIIIHDIFWTDPRDINTNKSSSYLDLAPLYGNSQEMQDSIRTFKDGRMKPDCYADKRLAGMPPGVSVLLIMFNRFHNHVAENLALINEGGRFNKPSDLLEGEAREAAWKKYDNDLFQVARLVTSGLYINITLVDYVRNIVNLNRVDTTWTLDPRQDAGAHVGTADGAERGTGNAVSAEFNLCYRWHSCISEKDSKFVEAQFQNIFGKPASEVRPDEMWKGFAKMEQNTPADPGQRTFGGFKRGPDGKFDDDDLVRCISEAVEDVAGAFGARNVPQAMKVVETMGIIQGRKWNVAGLNEFRKHFHLKPYSTFEDINSDPGVAEALRRLYDHPDNVELYPGLVAEEDKQPMVPGVGIAPTYTISRVVLSDAVCLVRGDRFYTTDFTPRNLTNWGYKEVDYDLSVNHGCVFYKLFIRAFPNHFKQNSVYAHYPMVVPSENKRILEALGRADLFDFEAPKYIPPRVNITSYGGAEYILETQEKYKVTWHEGLGFLMGEGGLKFMLSGDDPLHAQQRKCMAAQLYKDGWTEAVKAFYAGMMEELLVSKSYFLGNNKHRHVDIIRDVGNMVHVHFASQVFGLPLKTAKNPTGVFTEQEMYGILAAIFTTIFFDLDPSKSFPLRTKTREVCQKLAKLVEANVKLINKIPWSRGMFVGKPAKDEPLSIYGKTMIKGLKAHGLSDYDIAWSHVVPTSGAMVPNQAQVFAQAVDYYLSPAGMHYIPEIHMVALQPSTPETDALLLGYAMEGIRLAGTFGSYREAAVDDVVKEDNGRQVPVKAGDRVFVSFVDAARDPKHFPDPEVVNPRRPAKKYIHYGVGPHACLGRDASQIAITEMFRCLFRRRNVRRVPGPQGELKKVPRPGGFYVYMREDWGGLFPFPVTMRVMWDDE

SEQ ID NO: 59 - protein, 1161 aa, Glomerella cingulate; identical to SEQ ID NO: 52

SEQ ID NO: 60 - protein, 1283 aa, Fusarium oxysporum
MAEHKNGVATNGYEKKSSPASSSTKSEAKPLPNGDKKDGIVKSFKQLRVASKRPLPKEMGDGSYRVVENRPGLKQDIRRLRGRDLKTLLEIVKAKVKGETQQDDKTMIMERTIQLVANLSDHSKVQESLTNSFISQLWNSIDHPPMLYMGDKFRFRQPDGSNNNPYLPQLGAARTPYSRTVRPKGMSLGAQPDPEAIFESVFARDAFRKNPNNVSSILWYWATIIIHDLFWTNLQDPNQNDSSSYLDLAPLYGSTEKDRDSIRTFKDGQLKPDCFADKRLIGNPPGVPILLIMFNRFHNHVATNLADINEGGRFSKPAEHLSPEAADAAWKKRDTELFETARLVTSGLYINITLIDYVRNIINLNRVDTTWTLDPRQEMGVSVGTKDLSESGTGNVVSAEFNLCYRWHSCLSEMDDKWVQDFYTELLGENYGPMNLQTMMKALKAFEASVADEPSERTFGGFKRGPDGKFNDDELVEALATAIEQPGGAFGGRNVPRIMKPIEMLGIMRGRKWNLAGLNEFRKHFGLKAYETFEDINSDPSVADALRNLYQHPDYVELYPGIVAEEAKTPMVPGVGIAPTYTISRVVLSDAVALVRGDRYYTTDYNPRHLTNWGYKEVDYDLKVNHGCVFYKLFLRAFPQHFKGNSVYAHYPMVIPSENKKILTNIKRADRFDFSRPEPTATRINIIGYNAAKYILEDQQKYRVCWEEGLKHLMGEAGGRFMLSGDTALHAQQRKCMGKLLYNDTWRNAVKSFYATTAEKLLAEKSYRLAGKMQVDVVRDVGNVAHTHFVARMFNLPLKTSENPKGVFSEQELYMILAVIFVCIFFDIDPAKSFPLRQGAREVAQKLGGIIEMNVKLANSIGVKGLFTSKPDKNDDPLARYGENMAKGLKKAGLSTEDIVWSQILPTAGAMVPNQAQVFAQTLDWYLSPAGEKYRPELARIAALETGDETDALLLGYAMEGIRMAGTFGLYREATGPDTIHEDDGRSIPVNAGDRVFVSFVQAAQDPKIFPNPGVVDPKRPLDKYIHYGVGPHACLGRDISQVALTELFRAVFRKKGVRRVPGAQGELKKVPRPGGFFVYMTEDWGSIWPFPTSMKITWDDGCGTDLFTLLFWCRSVPWWDLLPETTQAAPFIISSFQSQQIYSPAEIAAVLALMAFESGDFQYKRNHYPGRPGQGTANMQMPNYNLLYAKSIPELAKGWQGIESVEGLSDQELGDLLDDVTVDKYNFGSGPWFLKTQCKEDVRQAFKTDVDTGFQKYIEECVGTDLQPRLEYFQRAKTAFGL

SEQ ID NO: 61 - protein, 1079 aa, Aspergillus fumigatus
MSEKQTGSANGGLGKTLAQLEQVVSASLRPLPSQTGDGTYVTEQVKTGILKDLSHVDLGDLKTLVDVSKSALTGEALDDRKYIMERVIQLSAGLPSTSQIGKELTNTFLTTLWNDLEHPPISYLGRDAMYRRADGSGNNVLWPHIGAAGTPYARSVQPKTVQSPNLPDPETLFDCLLARKEYKEHPNKISSVLFYIASIIIHDLFETDRKDPAISLTSSYLDLSPLYGNNQQEQDLIRTFKDGKLKPDCFSTKRVLGFPPGVGVVLIMFNRFHNYVVEKLAMINEGGRFTKPQESDTAAYAKYDNDLFQTGRLVTCGLYVNIILKDYVRTILNINRTDSIWSLDPRSEMKDGLLGRAAAQATGNQVAAEFNLVYRWHSCISQRDQKWTEDMYQELFPGQDPSKISLQDFLRGLGRWEAKLPGEPRERPFAGLQRKADGSYDDNDLVKIFEESVEDCAGAFGALHVPTVFRSIEALGIQQARSWNLATLNEFRKYFNLAPYKTFEEINSDPYVADQLKRLYDHPDRVEIYPGIIVEDAKESMAPGSGLCTNFTISRAILSDAVALVRGDRFHTVDFTPKHLTNWAYNEIQPQDSVDQTHVFYKLVLRAFPNHFRGDSIYAHFPLVVPSENKKILTKLGTADKYSWDRPNYTPPPQFINSHSACMSILSDQETFKVTWGSKIEFLMRHNNQPYGRDFMLSGDRTPNAMSRQMMGKALYRDKWETEVKRFYENITLKLLHRYSYKLAGVNQVDVVRDIANLAQVHFCASVFSLPLKTESNPRGIFTESELYQIMAVVFTSIFYDADIGKSFELNQAARAVTQQLGQLTLANVELIAKTGFIANLVNSLHRHDVLSEYGVHMIQRLLDSGMPAPEIVWTHVLPTAGGMVANQAQLFSQSLDYYLSEEGSVHLPEINRLAKEDTTEADDLLLRYFMEGARIRSSVALPRVVAQPTVVEDNGQKITLKQGQHIICNLVSASMDPVTFPEPDKVKLDRDMNLYAHFGFGPHQCLGLGLCKTALTTMLKVIGRLDNLRRAPGGQGKLKKLSGPGGIAMYMTPDQTAFFPFPTTMKIQWDGDLPEVKE

SEQ ID NO: 62 - protein, 1071 aa, Aspergillus terreus
MQGIGKAISQLEKVATASLRPLPTETGDGSYVAESTATGLVQDLPHVDLGDLKTLLDVTKNAATGEPIDDKGYVMERLIQLASGLPSTSRNAKQLTSAFLNQLWNDLDHPPVSTVGGEYSHRSADGSGNNILWPGIGAAGSHYARSVQPKTMQSPSLPDPEALFDSLLARKDFKEHPNKISSVLFYIASIIIHDLFQTDHRDSSINRTSSYLDLSPLYGNNQDEQYLMRTFKDGKLKPDCFSSKRILGFPPGVGVLLIMFNRFHNYVVEQLAAVNEGGRFTKPSESNDKEYAKYDNNLFQTGRLVTCGLYINIILKDYVRTILNINRTNSTWSLDPRMDMKDGLLGDAAPLATGNQVSAEFNLIYRWHSCISQRDEKWTTDLYNDIFSDKGQEDIPLNEFMMGVGKWEAGLPQQPAERPFAGLKRKPNGLFDDDDLVTIFKESVEDCAGAFGASHVPTIFKSIESLGIKQARAWNLATLNELRQYFGLTPHKTFEDINSDPYISEQLRRLYDHPDQVEIYPGVIVEETKESMLPGSGLCTNFTISRAILSDAVALVRGDRFYTVDYTPKQLTNWAFTEIQPKDSVDQGHMFHKLVYRAFPNYFKGNSVYAHFPMVVPSENQKILTALGSAEKYSWDKPGFIHPPQFINSHSTCVSILADQETFKVSWGDKIEFLMSNHDKIYGKDFMLSGDRLPNAESRKMMGAALYTDQWEEEVKKFYEKITLKLLKKHSYKIAGVNQVDIVRDVANLAQVNFCANVFSLPLKTEASPRGIFTESELYMIMAAVFAAIFYDADPANSFALNQAAREVTQQLGQVTMANVELIHKTGFISNLVNGLQRHDVLSNYGIHMIQRLLASGLPASEIVWTHLLPTAGGMVANQGQLFSQCLDYYLSEEGSVHLPEINRLAKENTPEADELLLRYFMEGARLRSSVGLPRVVAKPTVIDDNGTKLTLKEGQHILCNLVAASHDPVSFPEPEKVRLDRDMDLYVHFGSGPHKCLGFGLCKLGLTTMLKVVGGLDNLRRAPGPQGQLKRLAGPGGISKYMTADQSGFFPFPTTMKIQWDGDLPEPASD

SEQ ID NO: 63 - protein, 1080 aa, Aspergillus kawachii
MSGSNNHSIVNGIGSTISQVEKAISASLRPLPTATGNGTYVTEPAQTGIVKDLSHVDLTDFKALLEVVKDAVTGQPVDDRHYIMERVIQLAAGLPSTSKSGKDLTNTFLKQLWNDLEHPPISYLGRNTSYRKADGSGNNFLWPHIGAAGSHYARSVRPTTVQSPSLPDPSTLFESLLERKEYKEHPNKISSVLFYLASIIIHDLFQTDRNDYTLNKTSSYLDLSPLYGNNQDEQNLVRSFKDGKLKPDCFSSKRVLGFPPGVGVLLLMFNRFHNYVVENLATINEGGRFTKPDESDVDASTRYDNDLFQTGRLVTCGLYINIILKDYVRTILNINRTDSLWSLDPRADIQDSLLGSAPAEATGNQVSAEFNLVYRWHACVSQRDEKWTQDLYKDLFPGKDPNNVSLPEFLRGVAKWEASLPEQPPDRPFAGLQRNADGAFDDDDLANMFADGVEDCAGAFGAGNIPSVFRNIEALGILQARSWNLATLNEFRKFFDLAPYKTFEEINPDPYIAAQLKNLYDEPDLVEMYPGVIVEATKDAVVPGSGLCTNFTISRAILSDAVSLVRGDRFYTVDYTPKHLTNWAYHEIQPQDSVDQGQVFYKLVLRAFPNHFKGDSIYAHFPLVIPSENKKILEKLSVAQDYSWGRPSYTPTPQFISSNAACISVLNDQEAFKVTWGSKIEFLMRHNNHPYGRDFMLSGDKPPNAASRRMMGSALYRDKWESEVKRFYEDITIKLLRQHSYKLGGTNQVDIVRDVANYAQVHFCANVFSLPLKTESNPRGIFTEAELYEILALVFASIFYDADVGTSFQLNHTARDVTQQLGDLTMANVDFVNKAGFIANIVSSLHRHDVLSEYGEHMIQRLLHNNIPPADIVWTHLLPTAGGMVANQAQLFSQCLDYYLSDEGSVHLPDIKRLAQENTSEADSLLLRYFMEGARLRSSVGLPRLVAKPTVVDDGGSKYTLKPGQSVLCNLVSASMDPRSFPEPEKVKLDRDMSLYAHFGFGPHQCLGMGICKLALTTMLRVVGRLDNLRRAPGSQGQLKRIAGPGGISMYMTADQSSYWPFPSTMKIQWDGDLPSLATN

SEQ ID NO: 64 - protein, 1080 aa, Aspergillus clavatus
MSGKREESTNGGIGKTIAQIEKVVTASLRPLPSKTGDGTYVTEAVKTGLLKDLSHVDLGDLKTLLEVSKSALTGEAVDDKKYIMERVVQLAAGLPSTSQIGKDMTNTFLTTLWNDLEHPPISYLGRDAMYRKADGSGNNILWPHIGAAGTPYARSVRPKTMQSPNLPDPETLFDCLLARKEYKEHPNKISSVLFYIASIIIHDIFQTDRKDPTVSLTSSYLDLSPLYGNNQDEQNLVRTFKDGKLKPDCFSTKRVLGFPPGVGVLLIMFNRFHNHVVENLALINEGGRFTKPQESDAQAYAKYDNDLFQTGRLITCGLYVNIILKDYVRTILNINRTDSIWSLDPRADMKDGLLGEAAAQATGNQVSAEFNLVYRWHSCISKRDQKWTEDMYQEVFPGQDPSKLPLQDFMRGLGRWEAKLPGEPQERPFAGLQRKADGSYDDDDLVKIFGDSVEDCAGAFGVLHVPTVFRSIEALGIQQARSWNLATLNEFRNYFNLAPYKTFEEINPDPYVADQLRRLYDHPDRVEIYPGIIVEDTKESMAPGSGLCTNFTISRAILSDAVALVRGDRFHTVDFTPKHLTNWAYNEIQPQESVDQTHVLYKLVFRAFPNHFKGDSIYAHFPLVIPSENKKILTKLGTADKYSWDRPSFTHPPQFINSHSACMSILADQETFKVSWGKKIEFLMRHNDQPHGRDFMLSGDKPPNAESRQMMGKALYRNKWETEVKDFYEEITLKLLHRNSYKLAGTNQVDIVRDVANLAQVYFCASVFSLPLKTESNPRGVFTESELYQIMAVVFTSIFYDADVCKSFELNQGARAVTQQLGQLTMANVELIEKTGFIANLVNSLHRHDALTEYGVHMIQRLLDTGTPAAEIVWTHVLPTAGGMVANQAQLFSQCLDYYLSDEGSIHLPEINRLAKQDTPEADDLLLRYFMEGARLRSSVALPRVVAQPTVVEDNGQKVILKEGQHILCNLVSASMDPASFPEPDKVKLDRDMNLYAHFGFGPHQCLGIGLCKLALTTMLKVVGRLDNLRRAPGGQGRLKKLSGPGGIAMYMTPDQSGFFPFPTTMKIQWDGDLPPLKTE

SEQ ID NO: 65 - protein, 1080 aa, Aspergillus niger
MSGANNHSIVNGIGSTISQVEKAISASLRPLPTATGNGTYITEPDQTGIVKDLSHVDFTDIKALLEVIKDAVTGQPVDDRHYIMERVIQLAAGLPSTSKNGKDLTNAFLKQLWNDLEHPPISYLGRDSSYRKADGSGNNFLWPHIGAAGSHYARSVRPTTVQSPSLPDPSTLFASLLERKEYKEHPNKISSVLFYLASVIIHDLFQTDRSDFTLNKTSSYLDLSPLYGNNQDEQDLVRTFKDGKLKPDCFSSKRVLGFPPGVGVLLLMFNRFHNYVVENLATINEGGRFTKPDESDVDASTKYDNDLFQTGRLVTCGLYINIILKDYVRTILNINRTDSLWSLDPRADIQDSLLGSAPAEATGNQVSAEFNLVYRWHACISQRDEKWTQDLYKDLFPGKDPNNVSLQEFIRGVAKWEASLPEQPPDRPFAGLQRNADGAFDDGDLANMFADGVEDCAGAFGAGNIPSVFRNIEALGILQARSWNLATLNEFRKFFDLAPYKTFEEINPDPYIAAQLKNLYDEPDLVEMYPGVIVEATKDAIVPGSGLCTNFTISRAILSDAVSLVRGDRFYTVDYTPKHLTNWAYNEIQPQDSVDQGQVFYKLVLRAFPNHFKGDSVYAHFPLVIPSENKKILEKLSVAQDYSWGRPSYTPLPQFISSNAACISVLNDQEAFKVTWGSKIEFLMRHNNHPYGRDFMLSGDKPPNAASRRMMGSALYRDKWESEVKRFYEDITIKLLRQHSYQLGGVNQVDIVRDVANYAQVHFCANVFSLPLKTESNPRGIFAESELYEILALVFASIFYDADVGTSFQLNQTARDVTQQLGELTMANVDFVNKAGFIANLVSSLHRHDVLSEYGEHMIQRLLHSNVPPAEIVWTHLLPTAGGMVANQAQLFSQCLDYYLSDEGSIHLPDIKRLAKENTSEADALLLRYFMEGARLRSSVGLPRLVAKPTVVDDGGSKYTLKPGQSVLCNLVSASMDPRSFPEPEKVKLDRDMSLYAHFGFGPHQCLGMGICKLALTTMLRVVGRLDNLRRAPGSQGQLKKIAGPGGISMYMTADQSSYWPFPSTMKIQWDGDLPSLATN

SEQ ID NO: 66 - protein, 1127 aa, Glomerella cingulate
MSQQSHTEQFPKNQPPLAERLASARQLVTKAISAVPPHPEPLPSPNSDQGEPSNLLQDVKKLGFDDFDTLVHFFSSAVEGQINDNELLLENLIQLFAKLPQNSVKGKRLENGLINQLWNGIDHPPMTTLGEDHKYRAADGSGNAIHDPKMGAAGQPYARSTPAKSYQNPNQPEPEMIFDMLFARGGEFKPHPNKISSFMFYLATIITHDIFQTKNGTSPINQTSSYLDLAPLYGRNQAEQDLMRTKKNGLLKPDTFSSKRVLGFPPGVGTLLIMFNRYHNYVATNLATINEGGRFQKPTGDDPEKTAKYDNDLFQTARLITCGLYVSIILRDYVRTILGMNRTASSWALDPRTNEGKSILSQQTPEGTGNQVSVEFNLIYRWHNTISPKDEQWTKDVMKKVLGKDPTEMSLMEFGHAMRDWEQEIPDDPAQRGFMDLPRNADGTLNEADLAKIFKESVDDVAGSYGANRIPEVMRPIELMGIMASRSWNCATLNEFREHFGLTRHPTFEDINPDKEVAAKLRFLYGSPDAVELYPGLMAEKAKPPMAPGSGLCGNFTMTRAILSDAVALVRGDRFYTIDYTPKNLTNWGFNQASYDLNVDQSHVLYKLVFRAFPNSFQNNSIYAHFPFVIPSENKKILESIDKAYLYTWDEPKTKTPLIPILSHKAVSEVLYNQQDFKVITGDAINHLVAQPNKPHYGKDFCLSGDGKEHAKNRTLVRKSLISGPWETEIWKWYTHMTPKILNLNSFPIPGNKREIDLVRDVINVTNTRFNAALFCMPIKNEESPWGVYTDQELYSVLGALFQAVFMDADIGNSFKLRTIARELAQDLGKVVMLIAQTIKKAGLITDIVAKIREGEASLPTYGNHLIERMLSDGKDVEEVVWGTIMPVITANVANQSQVTSLCVDYYLDKEGKKHLPELYRLAHENTPEADETLLKYMLEGCRLRGPVAVYREATSTQVITDYSPCLPSESDPTGRDPITNPDIEGTKREVKIPRGYRVVCNFATAGRDPAIFEDPNEVRLDRPLDSYVHFGLGPHWCAGKEMSRVGQTSLFKQIVGLKNLRRAPGGRGEMKNFPASPWNGQVGLPVEGQNGSAAHQQPWLGLRAFMTVDQSSLWPIPTTMRVQWDE

SEQ ID NO: 67 - protein, 1165 aa, Gaeumannomyces graminis; identical to SEQ ID NO: 1

SEQ ID NO: 68 - protein, 1171 aa, Magnaporthe oryzae
MASSSSSGSSTRSSSPSDPPSSFFQKLGAFLGLFSKPQPPRPDYPHAPGNSAREEQTDITEDIQKLGFKDVETLLLYLNSSVKGVNDDKQLLLERLIQLLSKLPPTSTNGKKVTDGLITGLWESLDHPPVSSLGEKYRFREADGSNNNIHNPTLGVAGSHYARSAKPMVYQNPNPPAPETIFDTLMARDPAKFRPHPNQISSVLFYFATIITHDIFQTSSRDPSINLTSSYLDLSPLYGRNLEEQLSVRAMKDGLLKPDTFCSKRVHGFPPGVGVLLIMFNRFHNYVVTSLAKINEGNRFKKPVGDDTAAWEKYDNDLFQTGRLITCGLYVNIVLVDYVRTILNLNRVDSSWILDPRTEEGKSLLSKPTPEAVGNQVSVEFNLIYRWHCGMSQRDDKWTTDMLTEALGGKDPATATLPEFFGALGRFESSFPNEPEKRTLAGLKRQEDGSFEDEGLIKIMQESIEEVAGAFGPNHVPACMRAIEILGMNQARSWNVATLNEFREFIGLKRYDTFEDINPDPKVANLLAEFYGSPDAVELYPGINAEAPKPVIVPGSGLCPPSTTGRAILSDAVTLVRGDRFFTVDYTPRNLTNFGYQEAATDKSVDNGNVIYKLFFRAFPNHYAQNSIYAHFPFVIPSENKKIMESLGLADKYSWQPPQRKPATQMIRSHAAAVKILNNQKDFKVVWGESIGFLTKFPTGENPGLGFALAGDAPANQQSRDQLMKCIFSPKAWEDEVRQFCEATTWDLLRRYSAKVQDKGPHLKVHTHEIDVIRDVISLANARFFAAVYSLPLKTENGDDGVYSDHEMYRSLMLIFSAIFWDNDVSKSFKLRRDARAATQKLGALVEKHIVEMGSLFHSFKHSHSAVSDKTNGLANGGANGHANGNANGHTNGNGIHQNGGAAPSMLRSYGDLMLRRMIEAYGEGKSVKEAVYGQIMPSIAAGTANQTQIMAQCLDYYMSDDGAEHLPEMKRLASLETPEAFNTLMKYLFEGARIRNTTAVPRLVATDQTVEDNIPCLPDPKDSTFLRPIPNPQQAETTRTVKLSRGSMVLVDLTVAAHDATAFPDPEKVRLDRDLDSYTFFGLGPHRCAGDKVVRITMTAVFKVLLQLDGLRRAEGGRGVFKSLPASQWNGQAGRVAGEKPQWSGLRTYVNADESAFSQTPMNMKIRWDD

SEQ ID NO: 69 - protein, 1079 aa, Penicillium oxalicum
MVGHHGSETHGEKSPLVQIEQVFKAALRPLPTETGDGTYVKDTKLTGLAQDLSHVDLVDVKTLADVAKNAITGEAMNDREYIMERVIQLAAGLPTTSKNGRDLTNTFLSTLWNDLQHPPTSYLGRDSAYRQADGSGNNPFWPNIGAAGTPYARSVRPQTMQPGALPEPETLFDSLLARQKFKEHPNKISSVLFYLASIIIHDLFQTDPRNPTVSLSSSYLDLGPLYGNNQDEQNAVRTFKDGKLKPDCFSSKRILGFPPGVGVLLIMFNRFHNYVAEQLAQINEGGRFTKPAESNTKAYATWDNDLFQTSRLVTCGLYVNIILKDYVRTILNINRTDSTWSLDPRAEMKDGVLSHAAKQATGNQVSAEFNLVYRWHSCISARDQQWSEDLYRELFNGQDPNTLSTQQFIMGVGRWEGTLPQDPMERPFAKLQRQADGRFSDDDLVRFFEESVEDVAGAFGASNVPTVFRTIEVLGIKQARSWNLATLNEFRSFFNLQPYKTFEEINSDPYIADQLRHLYDHPDQVELYPGLVVEDAKEPMLPGSGLCTNYTTSRAILSDAVTLVRGDRFYTVDYTPKHLTNWAFNEISYDDSVDNGAIFYKLVLRAFPNHVRGDSVYAHFPMVVPSENKKILTSLGKSEKYSYSRPTYTPPPRMIKSHGACMSILADKETFKVTWGQKLEFILSRDGHSYGGDFMLSGDKAPHAQSRKMIGNALYRDQWKSEVRSFYESITLQLLRQKSYKLAGVNQVDIVRDVSNLAQIHFCANIFSLPLKTESNPHGVFTEQELYEIMALVFTCIFYDVEVTKSFQLEQASRQVAQQLGELVMANVDLVSKSGFVADIISRLRRHEHLTDYGVHMIQRLLDSGLPPKEIVWTHILPSASSMVANQAQLFIQCLDFYLKPENAHHLADIQRLSKEDTPESDELLLRYFMEGGRICSSVALPRVVAKSTVIEDNGEQVSLKEGEAIFLNLVSASHDPKAWPDPEEVRLDRDLNQYAHFGFGPHQCLGLGVCQVALPTMLRVVGQLQNLRRAPGLQGQLKKLPALGGLTMYMDADHSSISPYPSTMKIQWDGELPKARYT

SEQ ID NO: 70 - protein, 1074 aa, Penicillium chrysogenum
MAEKESNSSGKIAQLEQVVAAALRPLPTQTGDGSYVQEPTVTGLAKDLLNFDLKDAKTLADMAKTAVTGKAVNDRDYIMERVIQLASGLPSTSRNGKELTNTFLTQLWGDLEHPPISYLGRDAAYRKADGSGNNTFWPQIGAANTPYARSVRPKTMQPVALPEPEALFDSLLARKDFKEHPNKISSVLFHLASIIIHDLFQTDPRDQTKSLTSSYLDLSPLYGNNQKEQDTVRAFKDGKLKPDCFSTKRVLGFPPGVGVILIMFNRFHNSVVTQLAAINEGGRFTKPDESNAEAYATWDNDLFQTARLVTCGLYINIILKDYVRTILNVNRTDSLWSLDPRADIRDGLLGEAPAQATGNQVSAEFNLVYRWHSCVSSRDEKWSEDLYKEIFDGKDPKEISMQQFTGGLRQWESKLPADPQERPFAKLQRQADGKFDDNDLVKIFEESVEDPAGAFGALNVPDVFRGIEVLGIKQARSWNLATLNEFRQYFGLAAYQTFEEINPDPYVANQLKHFYDHPDLVELYPGLVVEETKQAMTPGSGLCTNFTTSRAILSDAVALVRGDRFYTVDFTPKHLTNWAFNEINNDVSVDGGQVFYKLILKAFPNHFRGDSVYAHFPLVVPDENKKILTSLGKVKTYSFDRPFYKAPPLFINSHSACTKILKDQEGFKVVWGEKIQFLMENSGRPYGRDFALSGDLPANAASRKMIGAALHRDKWESEVKAFYEDITLKLLERNSFKVAGVNQVDIVRDVAVLAQVNFCANVFSLSLKTESNPRGVFSEQELYQILAVIFASIFYDVDVSKSLQLCQTARNVAQQLGELTLANVELVAKTGFISNLVNRLHRHDILSEYGIHMIQRLLDSQLPVKDVVWSHILPTAGALVANQGQLFSQCIDYYLSEEAAEHLAEIQRLSREDTPEADELLVRYFMEGARLRCSVALPRFATKPTVVDDNGKRVTLKAGQEIICNLVVAGRDPVAFPDPDKVRLDRDMSLYTHFGFGPHECLGVKMCPLALSTMLKVLGRLDNVRRAPGPQGHLKRLDGLGGIAMYMDAEHSSFSPFPMTMKIQWDGDLPARRE

SEQ ID NO: 71 - protein, 1121 aa, Penicillium digitatum
MLRRISTQFKRSKDLKDSKDFKDSNGENTENSTEKNSKRASKVSPTRKSFSAKEEHHVVKRAEVVAVFEKFAQAIHASKEPLPNQTSDGAYLKHDKSSGLINDIKSLGFRELNTVKDLIASKASGELVDDKTYLMERIIQMVADLPGNSKNRTELTSLFLDELWNSIPHPPLSYMGDEYKYRSADGSNNNPTLPWLGAANTAYCRTIPPLTIQPSGLPDAGLIFDTLFARQEFTPHPNKVSSVFFDWASLIIHDIFQTDYRQQHLNKTSAYLDLSILYGDVQEQQDLIRSHQDGKLKPDCFSEGRLQALPAACGVLLVMLNRFHNHVVTQLAEINENGRFSKPRPGLSEEDAKKVWTKRDEDLFQTGRLITCGLYINITLYDYLRTIVNLNRTNSTWCLDPRAQVEKAGATPSGLGNQCSVEFNLAYRWHSTISQGDEKWIEQIYHDLMGKPAEEVTMPELLMGLKKVEGLLDTDPAKRTFARLQRNEDGFFNDGELVNILTHATEDVASSFGPRNVPKAMRSIEILGIEASRRWNVGSLNEFRKHFGLKPYETFEEVNSNPEISNTLRHLYDHPDFIELYPGIVTEEAKEPMIPGVGIAPTYTISRAVLSDAVALVRGDRHYTIDYNPRNLTNWGYNECRYDLNINQGCIFYKLATRAFPNHYRPDSIYAHYPMTIPSENRNIMKDLGREQDYSWDKPAFIEPRVNLASHQNAKLLLENQRDFRPSWARSVSELFGKGEFDTKQREAIGKALNTEDFPKLVKTFYEDITERLIVEKGGQLGKINQIDITRDVGNLAHVHFASTIFGIPLKTEQSPQGLFTEHEMYMILSTIFSALFFDVDAPRSYALNHAASAVSTQLGQVVEATVKADTNSGLFSGIMDSFRPHDNALREFGTEAVRRMKEAGSSASDITWSAIIPTIVGLVPSQGQVFTQIIEFYTAPENQAHLAAIHSLTKTDSAESDEKLHRYCLEAIRLNGTFGAFREAKEAVTIEEDGKVYAVQPGQQVFASFNQANHDPSVFPEPYQVNLHRPLNSYINHGQGPTTGFGEQITKIALVAMLRVVGRLQGLRRAAGAQGQLQKIPQEGGYYVYLRGDGAAYCPFPMSLKLHWDGPVGQKKTPSS

SEQ ID NO: 72 - protein, 805 aa, Acaryochloris marina; identical to SEQ ID NO: 3

SEQ ID NO: 73 - protein, 822 aa, Nostoc sp.
MTNEIQNPVDHLVGDPRVRDIEPKFSKIISDIARVFGQMAQLKGRRATHSFGTVAKGVLEVVKQPDIPPHRLLEAGKKFPVLLRHANIKGFRDDAILDGRGATLRILNGPADAPITALDLHTPILDVLMSTGRCFILPDAASFSRWVASPLQDRAKLLVEFPKITPIFAEIIRNPDSYTKLHYYSETTYLFIGLDGKQYYLRYRLINSDRSADTGFINSADLRLPLDYLPRLEDDTRPETYLQNDYQQKVKNGGVKYILQFQLRAVSDNQAANEEAKDCTIPWDETQYPCKDVAVISLTEIVPSELAEPLEFNPYHAPPDLSLILAHSINETASVNHLRSVVYQISANMRKFQQPSAELVDWGIKGNQPDPKQVYTYYGQIGQDIPRYDFRRPLPDRVKPKPRYIANFGLHLFPARPLGSIPMLGIVGVAETMQALGQTAPQWMPANLTRTRPDKYEDQFFVERRLNGFNPGKFNRVHTFEPWQYTIRYDCRKYKVEEAGILPAEIEARFKFEDHNLHLHSIKFILNGKTETHKPGDADWEWSKRLFRTAEFVFQEIQSHLGRTHMNLDQYAMAYYRNVVNNPIRLLLEPHFDGLLNINSLGAALILGATGFIPEASSLSPEEVDIVLKDEISRLSYRNWSPHIQALKDEVQNNHFDRAALSVWEAIEEYVSEFFQKQEAGIKAYWSEIGGMSEDLVKHSVLGQKSQSLAIANINDLKQLCIYVIYLSSFFHSWVNNKQYDDGGDPAYASIGLWDGHNPQYNPITVAEKHARQVTLLWTLSSVRYNPVMEVGPPALKDRLWKRRKIIQPGIPVESIMMSTNI

SEQ ID NO: 74 - protein, 371 aa, Agrocybe aegerita
MKYFPLFPTLVFAARVVAFPAYASLAGLSQQELDAIIPTLEAREPGLPPGPLENSSAKLVNDEAHPWKPLRPGDIRGPCPGLNTLASHGYLPRNGVATPVQIINAVQEGLNFDNQAAVFATYAAHLVDGNLITDLLSIGRKTRLTGPDPPPPASVGGLNEHGTFEGDASMTRGDAFFGNNHDFNETLFEQLVDYSNRFGGGKYNLTVAGELRFKRIQDSIATNPNFSFVDFRFFTAYGETTFPANLFVDGRRDDGQLDMDAARSFFQFSRMPDDFFRAPSPRSGTGVEVVIQAHPMQPGRNVGKINSYTVDPTSSDFSTPCLMYEKFVNITVKSLYPNPTVQLRKALNTNLDFFFQGVAAGCTQVFPYGRD

SEQ ID NO: 75 - protein, 417 aa, Bacillus subtilis
MNEQIPHDKSLDNSLTLLKEGYLFIKNRTERYNSDLFQARLLGKNFICMTGAEAAKVFYDTDRFQRQNALPKRVQKSLFGVNAIQGMDGSAHIHRKMLFLSLMTPPHQKRLAELMTEEWKAAVTRWEKADEVVLFEEAKEILCRVACYWAGVPLKETEVKERADDFIDMVDAFGAVGPRHWKGRRARPRAEEWIEVMIEDARAGLLKTTSGTALHEMAFHTQEDGSQLDSRMAAIELINVLRPIVAISYFLVFSALALHEHPKYKEWLRSGNSREREMFVQEVRRYYPFGPFLGALVKKDFVWNNCEFKKGTSVLLDLYGTNHDPRLWDHPDEFRPERFAEREENLFDMIPQGGGHAEKGHRCPGEGITIEVMKASLDFLVHQIEYDVPEQSLHYSLARMPSLPESGFVMSGIRRKS

SEQ ID NO: 76 - protein, 415 aa, Sphingomonas paucimobilis
MPKTPHTKGPDETLSLLADPYRFISRQCQRLGANAFESRFLLKKTNCLKGAKAAEIFYDTTRFEREGAMPVAIQKTLLGQGGVQGLDGETHRHRKQMFMGLMTPERVRALAQLFEAEWRRAVPGWTRKGEIVFYDELHEPLTRAVCAWAGVPLPDDEAGNRAGELRALFDAAGSASPRHLWSRLARRRVDAWAKRIIEGIRAGSIGSGSGTAAYAIAWHRDRHDDLLSPHVAAVELVNVLRPTVAIAVYITFVAHALQTCSGIRAALVQQPDYAELFVQEVRRFYPFFPAVVARASQDFEWEGMAFPEGRQVVLDLYGSNHDAATWADPQEFRPERFRAWDEDSFNFIPQGGGDHYLGHRCPGEWIVLAIMKVAAHLLVNAMRYDVPDQDLSIDFARLPALPKSGFVMRNVHIGG

SEQ ID NO: 77 - protein, 418 aa, Clostridium acetobutylicum
MLLKENTAKDKGIDSTLDLLKEGYLFIKNRADHYQSDLFETRLMGQRIICMTGEEAARIFYDSDKFKRQGAAPKRVQETLLGENAIQTLDGESHLHRKKLFMLLTNQVQQKRLAELTTEKWEASASKWHTKSIVLFNEANEILCQVACHWAGVPLMESDIKNRAEDFSSMIDSFGAVGPRHWKGKKARNTIEAWIKEIIENVRSGRIRAEEGSPLHEIAFYIDVNGQQMPAEMAAIELINILRPIVAISTFITFSALALYEHSEYREKLQSKDIRYLEMFTQEVRRYYPFAPFVGARVRKDFLWNNCEFKKEMLVLLDIYGTNHDSRIWQKPYEFIPDRFRSYKGNLFDFIPQGGGDPSSTHRCPGEGITLEIMKTSLDFLSTKIDFTVPDQDLSYSLSKIPTLPKSGFIIDNINLKL

SEQ ID NO: 78 - protein, 646 aa, Elizabethkingia meningoseptica
MNPITSKFDKVLNASSEYGHVNHEPDSSKEQQRNTPQKSMPFSDQIGNYQRNKGIPVQSYDNSKIYIIGSGIAGMSAAYYFIRDGHVPAKNITFLEQLHIDGGSLDGAGNPTDGYIIRGGREMDMTYENLWDMFQDIPALEMPAPYSVLDEYRLINDNDSNYSKARLINNKGEIKDFSKFGLNKMDQLAIIRLLLKNKEELDDLTIEDYFSESFLKSNFWTFWRTMFAFENWHSLLELKLYMHRFLHAIDGLNDLSSLVFPKYNQYDTFVTPLRKFLQEKGVNIHLNTLVKDLDIHINTEGKVVEGIITEQDGKEVKIPVGKNDYVIVTTGSMTEDTFYGNNKTAPIIGIDNSTSGQSAGWKLWKNLAAKSEIFGKPEKFCSNIEKSAWESATLTCKPSALIDKLKEYSVNDPYSGKTVTGGIITITDSNWLMSFTCNRQPHFPEQPDDVLVLWVYALFMDKEGNYIKKTMLECTGDEILAELCYHLGIEDQLENVQKNTIVRTAFMPYITSMFMPRAKGDRPRVVPEGCKNLGLVGQFVETNNDVVFTMESSVRTARIAVYKLLNLNKQVPDINPLQYDIRHLLKAAKTLNDDKPFVGEGLLRKVLKGTYFEHVLPAGAAEEEEHESFIAEHVNKFREWVKGIRG

SEQ ID NO: 79 - protein, 589 aa, Macrococcus caseolyticus
MYYSNGNYEAFARPKKPEGVDNKSAYLVGSGLASLAAASFLIRDGQMKGENIHILEELDLPGGSLDGILNPERGYIMRGGREMENHFECLWDLFRSVPSLEVEDASVLDEFYWLNKEDPNYSKCRVIENRGQRLESDGKMTLTKKANKEIIQLCLMKEEQLNDVKISDVFSKDFLDSNFWIYWKTMFAFEPWHSAMEMRRYLMRFIHHIGGLADFSALKFTKFNQFESLVMPLIEHLKAKNVTFEYGVTVKNIQVECSKESKVAKAIDIVRRGNEESIPLTENDLVFVTNGSITESTTYGDNDTPAPPTSKPGGAWQLWENLSTQCEEFGNPAKFYKDLPEKSWFVSATATTNNKEVIDYIQKICKRDPLSGRTVTGGIVTVDDSNWQLSFTLNRQQQFKNQPDDQVSVWIYALYSDERGERTNKTIVECSGKEICEEWLYHMGVPEEKISALAAECNTIPSYMPYITAYFMPRKEGDRPLVVPHGSKNIAFIGNFAETERDTVFTTEYSVRTAMEAVYKLLEVDRGVPEVFASVYDVRILLHALSVLNDGKKLDEIDMPFYERLVEKRLLKKASGTFIEELLEEANLI

SEQ ID NO: 80 - protein, 590 aa, Streptococcus pyogenes
MYYTSGNYEAFATPRKPEGVDQKSAYIVGTGLAGLAAAVFLIRDGHMAGERIHLFEELPLAGGSLDGIEKPHLGFVTRGGREMENHFECMWDMYRSIPSLEIPGASYLDEFYWLDKDDPNSSNCRLIHKRGNRVDDDGQYTLGKQSKELIHLIMKTEESLGDQTIEEFFSEDFFKSNFWVYWATMFAFEKWHSAVEMRRYAMRFIHHIDGLPDFTSLKFNKYNQYDSMVKPIIAYLESHDVDIQFDTKVTDIQVEQTAGKKVAKTIHMTVSGEAKAIELTPDDLVFVTNGSITESSTYGSHHEVAKPTKALGGSWNLWENLAAQSDDFGHPKVFYQDLPAESWFVSATATIKHPAIEPYIERLTHRDLHDGKVNTGGIITITDSNWMMSFAIHRQPHFKEQKENETTVWIYGLYSNSEGNYVHKKIEECTGQEITEEWLYHLGVPVDKIKDLASQEYINTVPVYMPYITSYFMPRVKGDRPKVIPDGSVNLAFIGNFAESPSRDTVFTTEYSIRTAMEAVYSFLNGERGIPQGFNSAYDIRELLKAFYYLNDKKAIKDMDLPIPALIEKIGHKKIKDTFIEELLKDANLM